European Patent Specification EP 3 842 542 B1, published June 24, 2026. Title: MASSIVELY PARALLEL SINGLE CELL ANALYSIS. Applicant: CELLULAR RESEARCH, INC. Application PCT/US2014/053301. The sequence listing filed with the application follows.

SEQUENCE LISTING (843 sequences)

SEQ ID NO: 1 - DNA, 18 bp, Artificial Sequence
  source: /note="Description of Artificial Sequence: Synthetic primer"
  misc_feature (1)..(18): /note="This sequence may encompass 12-18 nucleotides"
tttttttttttttttttt

SEQ ID NO: 2 - DNA, 20 bp, Artificial Sequence
  source: /note="Description of Artificial Sequence: Synthetic primer"
cccctggaagaagatgatga

SEQ ID NO: 3 - DNA, 42 bp, Artificial Sequence
  source: /note="Description of Artificial Sequence: Synthetic primer"
cagacgtgtgctcttccgatctttctccaacaagttgcctcc

SEQ ID NO: 4 - DNA, 21 bp, Artificial Sequence
  source: /note="Description of Artificial Sequence: Synthetic primer"
gaggaaatgaagccaaacaca

SEQ ID NO: 5 - DNA, 42 bp, Artificial Sequence
  source: /note="Description of Artificial Sequence: Synthetic primer"
cagacgtgtgctcttccgatctaatcgtgaccttaaaggccc

SEQ ID NO: 6 - DNA, 20 bp, Artificial Sequence
  source: /note="Description of Artificial Sequence: Synthetic primer"
ttagccacctcatgcctttc

SEQ ID NO: 7 - DNA, 41 bp, Artificial Sequence
  source: /note="Description of Artificial Sequence: Synthetic primer"
cagacgtgtgctcttccgatctctactgtggtggctccgct

SEQ ID NO: 8 - DNA, 20 bp, Artificial Sequence
  source: /note="Description of Artificial Sequence: Synthetic primer"
ggaggaggattgtgctgatg

SEQ ID NO: 9 - DNA, 45 bp, Artificial Sequence
  source: /note="Description of Artificial Sequence: Synthetic primer"
cagacgtgtgctcttccgatctgtgtccgcataagaaaaagaatc

SEQ ID NO: 10 - DNA, 20 bp, Artificial Sequence
  source: /note="Description of Artificial Sequence: Synthetic primer"
gcaagaaggtgctgacttcc

SEQ ID NO: 11 - DNA, 42 bp, Artificial Sequence
  source: /note="Description of Artificial Sequence: Synthetic primer"
cagacgtgtgctcttccgatctctgcatgtggatcctgagaa

SEQ ID NO: 12 - DNA, 20 bp, Artificial Sequence
  source: /note="Description of Artificial Sequence: Synthetic primer"
ctgcagtcccatcctcttgt

SEQ ID NO: 13 - DNA, 42 bp, Artificial Sequence
  source: /note="Description of Artificial Sequence: Synthetic primer"
cagacgtgtgctcttccgatctgatgaggtggagagtgggaa

SEQ ID NO: 14 - DNA, 22 bp, Artificial Sequence
  source: /note="Description of Artificial Sequence: Synthetic primer"
ggacataacagacttggaagca

SEQ ID NO: 15 - DNA, 46 bp, Artificial Sequence
  source: /note="Description of Artificial Sequence: Synthetic primer"
cagacgtgtgctcttccgatctcaatccattttgtaactgaacctt

SEQ ID NO: 16 - DNA, 19 bp, Artificial Sequence
  source: /note="Description of Artificial Sequence: Synthetic primer"
aagcctctgggtcagtggt

SEQ ID NO: 17 - DNA, 43 bp, Artificial Sequence
  source: /note="Description of Artificial Sequence: Synthetic primer"
cagacgtgtgctcttccgatcttggaaaagggatagaggttgg

SEQ ID NO: 18 - DNA, 20 bp, Artificial Sequence
  source: /note="Description of Artificial Sequence: Synthetic primer"
tagacagatccccgttcctg

SEQ ID NO: 19 - DNA, 42 bp, Artificial Sequence
  source: /note="Description of Artificial Sequence: Synthetic primer"
cagacgtgtgctcttccgatctacagggagaagggataaccc

SEQ ID NO: 20 - DNA, 18 bp, Artificial Sequence
  source: /note="Description of Artificial Sequence: Synthetic primer"
cagcatcccagccttgag

SEQ ID NO: 21 - DNA, 42 bp, Artificial Sequence
  source: /note="Description of Artificial Sequence: Synthetic primer"
cagacgtgtgctcttccgatctcctcaatggccttttgctac

SEQ ID NO: 22 - DNA, 20 bp, Artificial Sequence
  source: /note="Description of Artificial Sequence: Synthetic primer"
cctctaaactgccccacctc

SEQ ID NO: 23 - DNA, 42 bp, Artificial Sequence
  source: /note="Description of Artificial Sequence: Synthetic primer"
cagacgtgtgctcttccgatctccttaatcgctgcctctagg

SEQ ID NO: 24 - DNA, 21 bp, Artificial Sequence
  source: /note="Description of Artificial Sequence: Synthetic primer"
  source: /note="Description of Combined DNA/RNA Molecule: Synthetic primer"
cacatggccuccaaggaguaa

SEQ ID NO: 25 - DNA, 42 bp, Artificial Sequence
  source: /note="Description of Artificial Sequence: Synthetic primer"
cagacgtgtgctcttccgatctcagcaagagcacaagaggaa

SEQ ID NO: 26 - DNA, 19 bp, Artificial Sequence
  source: /note="Description of Artificial Sequence: Synthetic primer"
gcagggtcccagtcctatg

SEQ ID NO: 27 - DNA, 42 bp, Artificial Sequence
  source: /note="Description of Artificial Sequence: Synthetic primer"
cagacgtgtgctcttccgatctccaatcatgaggaagatgca

SEQ ID NO: 28 - DNA, 20 bp, Artificial Sequence
  source: /note="Description of Artificial Sequence: Synthetic primer"
tccaggaggattaccgaaaa

SEQ ID NO: 29 - DNA, 42 bp, Artificial Sequence
  source: /note="Description of Artificial Sequence: Synthetic primer"
cagacgtgtgctcttccgatctccatccaagggagagtgaga

SEQ ID NO: 30 - DNA, 20 bp, Artificial Sequence
  source: /note="Description of Artificial Sequence: Synthetic primer"
aatggcaaaggaaggtggat

SEQ ID NO: 31 - DNA, 42 bp, Artificial Sequence
  source: /note="Description of Artificial Sequence: Synthetic primer"
cagacgtgtgctcttccgatctgcagacaccttggacatcct

SEQ ID NO: 32 - DNA, 20 bp, Artificial Sequence
  source: /note="Description of Artificial Sequence: Synthetic primer"
agatctgagccagtcgctgt

SEQ ID NO: 33 - DNA, 43 bp, Artificial Sequence
  source: /note="Description of Artificial Sequence: Synthetic primer"
cagacgtgtgctcttccgatcttggtgcagagctgaagatttt

SEQ ID NO: 34 - DNA, 20 bp, Artificial Sequence
  source: /note="Description of Artificial Sequence: Synthetic primer"
aaaagtgggcttgattctgc

SEQ ID NO: 35 - DNA, 42 bp, Artificial Sequence
  source: /note="Description of Artificial Sequence: Synthetic primer"
cagacgtgtgctcttccgatctttttgttcgcatggtcacac

SEQ ID NO: 36 - DNA, 20 bp, Artificial Sequence
  source: /note="Description of Artificial Sequence: Synthetic primer"
atattcctttgggcctctgc

SEQ ID NO: 37 - DNA, 42 bp, Artificial Sequence
  source: /note="Description of Artificial Sequence: Synthetic primer"
cagacgtgtgctcttccgatcttcaagtttgggtctgtgctg

SEQ ID NO: 38 - DNA, 20 bp, Artificial Sequence
  source: /note="Description of Artificial Sequence: Synthetic primer"
cccccgaaaatgttcaataa

SEQ ID NO: 39 - DNA, 41 bp, Artificial Sequence
  source: /note="Description of Artificial Sequence: Synthetic primer"
cagacgtgtgctcttccgatcttgctcttgtcataccccca

SEQ ID NO: 40 - DNA, 20 bp, Artificial Sequence
  source: /note="Description of Artificial Sequence: Synthetic primer"
tagcttcctcctctggtggt

SEQ ID NO: 41 - DNA, 44 bp, Artificial Sequence
  source: /note="Description of Artificial Sequence: Synthetic primer"
cagacgtgtgctcttccgatcttttgcctttccataatcactca

SEQ ID NO: 42 - DNA, 20 bp, Artificial Sequence
  source: /note="Description of Artificial Sequence: Synthetic primer"
ctggctctccccaatatcct

SEQ ID NO: 43 - DNA, 42 bp, Artificial Sequence
  source: /note="Description of Artificial Sequence: Synthetic primer"
cagacgtgtgctcttccgatctgctctgaggactgcaccatt

SEQ ID NO: 44 - DNA, 20 bp, Artificial Sequence
  source: /note="Description of Artificial Sequence: Synthetic primer"
gtggtgttggggtatggttt

SEQ ID NO: 45 - DNA, 42 bp, Artificial Sequence
  source: /note="Description of Artificial Sequence: Synthetic primer"
cagacgtgtgctcttccgatctatacacagatgcccattgca

SEQ ID NO: 46 - DNA, 20 bp, Artificial Sequence
  source: /note="Description of Artificial Sequence: Synthetic primer"
agacaggtccttttcgatgg

SEQ ID NO: 47 - DNA, 42 bp, Artificial Sequence
  source: /note="Description of Artificial Sequence: Synthetic primer"
cagacgtgtgctcttccgatcttgtgcaatatgtgatgtggc

SEQ ID NO: 48 - DNA, 22 bp, Artificial Sequence
  source: /note="Description of Artificial Sequence: Synthetic primer"
ttgagacaggcacatacagctt

SEQ ID NO: 49 - DNA, 42 bp, Artificial Sequence
  source: /note="Description of Artificial Sequence: Synthetic primer"
cagacgtgtgctcttccgatctttgcttcctcaatctgtcca

SEQ ID NO: 50 - DNA, 20 bp, Artificial Sequence
  source: /note="Description of Artificial Sequence: Synthetic primer"
ccccaaccacttcattcttg

SEQ ID NO: 51 - DNA, 43 bp, Artificial Sequence
  source: /note="Description of Artificial Sequence: Synthetic primer"
cagacgtgtgctcttccgatctttcaattcctctgggaatgtt

SEQ ID NO: 52 - DNA, 20 bp, Artificial Sequence
  source: /note="Description of Artificial Sequence: Synthetic primer"
tgcctagaggtgctcattca

SEQ ID NO: 53 - DNA, 42 bp, Artificial Sequence
  source: /note="Description of Artificial Sequence: Synthetic primer"
cagacgtgtgctcttccgatctgttgatgctggaggcagaat

SEQ ID NO: 54 - DNA, 20 bp, Artificial Sequence
  source: /note="Description of Artificial Sequence: Synthetic primer"
agcctgggtcacagatcaag

SEQ ID NO: 55 - DNA, 42 bp, Artificial Sequence
  source: /note="Description of Artificial Sequence: Synthetic primer"
cagacgtgtgctcttccgatctaggtaggagggtggatggag

SEQ ID NO: 56 - DNA, 20 bp, Artificial Sequence
  source: /note="Description of Artificial Sequence: Synthetic primer"
ccagcaccagggagtttcta

SEQ ID NO: 57 - DNA, 42 bp, Artificial Sequence
  source: /note="Description of Artificial Sequence: Synthetic primer"
cagacgtgtgctcttccgatctaggaaaggattggaacagca

SEQ ID NO: 58 - DNA, 20 bp, Artificial Sequence
  source: /note="Description of Artificial Sequence: Synthetic primer"
gggtttcaggttccaatcag

SEQ ID NO: 59 - DNA, 43 bp, Artificial Sequence
  source: /note="Description of Artificial Sequence: Synthetic primer"
cagacgtgtgctcttccgatcttttgtaactttttgcaaggca

SEQ ID NO: 60 - DNA, 20 bp, Artificial Sequence
  source: /note="Description of Artificial Sequence: Synthetic primer"
gtgaggagtgggtccagaaa

SEQ ID NO: 61 - DNA, 40 bp, Artificial Sequence
  source: /note="Description of Artificial Sequence: Synthetic primer"
cagacgtgtgctcttccgatctagtggggaggagcaggag

SEQ ID NO: 62 - DNA, 20 bp, Artificial Sequence
  source: /note="Description of Artificial Sequence: Synthetic primer"
ccattcccttcttcctcctc

SEQ ID NO: 63 - DNA, 42 bp, Artificial Sequence
  source: /note="Description of Artificial Sequence: Synthetic primer"
cagacgtgtgctcttccgatcttacctacaagatcccgcgtc

SEQ ID NO: 64 - DNA, 20 bp, Artificial Sequence
  source: /note="Description of Artificial Sequence: Synthetic primer"
ttggacatagcccaagaaca

SEQ ID NO: 65 - DNA, 42 bp, Artificial Sequence
  source: /note="Description of Artificial Sequence: Synthetic primer"
cagacgtgtgctcttccgatcttgtgcctcactggacttgtc

SEQ ID NO: 66 - DNA, 20 bp, Artificial Sequence
  source: /note="Description of Artificial Sequence: Synthetic primer"
acctgaagctgaatgcctga

SEQ ID NO: 67 - DNA, 42 bp, Artificial Sequence
  source: /note="Description of Artificial Sequence: Synthetic primer"
cagacgtgtgctcttccgatctctggaggccacctcttctaa

SEQ ID NO: 68 - DNA, 19 bp, Artificial Sequence
  source: /note="Description of Artificial Sequence: Synthetic primer"
ggtaaacacgcctgcaaac

SEQ ID NO: 69 - DNA, 42 bp, Artificial Sequence
  source: /note="Description of Artificial Sequence: Synthetic primer"
cagacgtgtgctcttccgatctcaggactcagaagcctctgg

SEQ ID NO: 70 - DNA, 24 bp, Artificial Sequence
  source: /note="Description of Artificial Sequence: Synthetic primer"
caacaaagcacagtgttaaatgaa

SEQ ID NO: 71 - DNA, 42 bp, Artificial Sequence
  source: /note="Description of Artificial Sequence: Synthetic primer"
cagacgtgtgctcttccgatcttgtgtcagctactgcggaaa

SEQ ID NO: 72 - DNA, 20 bp, Artificial Sequence
  source: /note="Description of Artificial Sequence: Synthetic primer"
tgagcagatccacaggaaaa

SEQ ID NO: 73 - DNA, 44 bp, Artificial Sequence
  source: /note="Description of Artificial Sequence: Synthetic primer"
cagacgtgtgctcttccgatctgaaatggagtctcaaagcttca

SEQ ID NO: 74 - DNA, 20 bp, Artificial Sequence
  source: /note="Description of Artificial Sequence: Synthetic primer"
tcccaactacgctgatttga

SEQ ID NO: 75 - DNA, 42 bp, Artificial Sequence
  source: /note="Description of Artificial Sequence: Synthetic primer"
cagacgtgtgctcttccgatctgaccaaaaggaatgtgtggg

SEQ ID NO: 76 - DNA, 21 bp, Artificial Sequence
  source: /note="Description of Artificial Sequence: Synthetic primer"
tgcaagagtgacagtggattg

SEQ ID NO: 77 - DNA, 43 bp, Artificial Sequence
  source: /note="Description of Artificial Sequence: Synthetic primer"
cagacgtgtgctcttccgatcttcaaccaaggtttgcttttgt

SEQ ID NO: 78 - DNA, 20 bp, Artificial Sequence
  source: /note="Description of Artificial Sequence: Synthetic primer"
agaggctgaaagaggccaat

SEQ ID NO: 79 - DNA, 43 bp, Artificial Sequence
  source: /note="Description of Artificial Sequence: Synthetic primer"
cagacgtgtgctcttccgatctaatatgggttgcatttggtca

SEQ ID NO: 80 - DNA, 23 bp, Artificial Sequence
  source: /note="Description of Artificial Sequence: Synthetic primer"
aaatctgcagaaggaaaaatgtg

SEQ ID NO: 81 - DNA, 42 bp, Artificial Sequence
  source: /note="Description of Artificial Sequence: Synthetic primer"
cagacgtgtgctcttccgatctagttttcaatgatgggcgag

SEQ ID NO: 82 - DNA, 20 bp, Artificial Sequence
  source: /note="Description of Artificial Sequence: Synthetic primer"
gctcaagggagagctgaaga

SEQ ID NO: 83 - DNA, 42 bp, Artificial Sequence
  source: /note="Description of Artificial Sequence: Synthetic primer"
cagacgtgtgctcttccgatctgactacctgcccccagagat

SEQ ID NO: 84 - DNA, 20 bp, Artificial Sequence
  source: /note="Description of Artificial Sequence: Synthetic primer"
gtggcgtgtatgagtggaga

SEQ ID NO: 85 - DNA, 41 bp, Artificial Sequence
  source: /note="Description of Artificial Sequence: Synthetic primer"
cagacgtgtgctcttccgatctcactcgcccagagactcag

SEQ ID NO: 86 - DNA, 20 bp, Artificial Sequence
  source: /note="Description of Artificial Sequence: Synthetic primer"
gcacatctcatggcagctaa

SEQ ID NO: 87 - DNA, 42 bp, Artificial Sequence
  source: /note="Description of Artificial Sequence: Synthetic primer"
cagacgtgtgctcttccgatctgcttcacaaaccttgctcct

SEQ ID NO: 88 - DNA, 20 bp, Artificial Sequence
  source: /note="Description of Artificial Sequence: Synthetic primer"
acattttctgccacccaaac

SEQ ID NO: 89 - DNA, 42 bp, Artificial Sequence
  source: /note="Description of Artificial Sequence: Synthetic primer"
cagacgtgtgctcttccgatctaacagcaccctctccagatg

SEQ ID NO: 90 - DNA, 21 bp, Artificial Sequence
  source: /note="Description of Artificial Sequence: Synthetic primer"
gcctggtagaattggcttttc

SEQ ID NO: 91 - DNA, 45 bp, Artificial Sequence
  source: /note="Description of Artificial Sequence: Synthetic primer"
cagacgtgtgctcttccgatctttttgtagccaacattcattcaa

SEQ ID NO: 92 - DNA, 20 bp, Artificial Sequence
  source: /note="Description of Artificial Sequence: Synthetic primer"
caattggcagccctatttca

SEQ ID NO: 93 - DNA, 42 bp, Artificial Sequence
  source: /note="Description of Artificial Sequence: Synthetic primer"
cagacgtgtgctcttccgatctgttcagcagactggtttgca

SEQ ID NO: 94 - DNA, 20 bp, Artificial Sequence
  source: /note="Description of Artificial Sequence: Synthetic primer"
ccgtgaggatgtcactcaga

SEQ ID NO: 95 - DNA, 42 bp, Artificial Sequence
  source: /note="Description of Artificial Sequence: Synthetic primer"
cagacgtgtgctcttccgatctacgaggaagccctaagacgt

SEQ ID NO: 96 - DNA, 20 bp, Artificial Sequence
  source: /note="Description of Artificial Sequence: Synthetic primer"
ttgagcctggggtgtaagac

SEQ ID NO: 97 - DNA, 42 bp, Artificial Sequence
  source: /note="Description of Artificial Sequence: Synthetic primer"
cagacgtgtgctcttccgatctgtcttccaggattcacggtg

SEQ ID NO: 98 - DNA, 20 bp, Artificial Sequence
  source: /note="Description of Artificial Sequence: Synthetic primer"
gagcacctcctggaagattg

SEQ ID NO: 99 - DNA, 42 bp, Artificial Sequence
  source: /note="Description of Artificial Sequence: Synthetic primer"
cagacgtgtgctcttccgatcttaagcaccagtgggactgtg

SEQ ID NO: 100 - DNA, 20 bp, Artificial Sequence
  source: /note="Description of Artificial Sequence: Synthetic primer"
taggagcaggcctgagaaaa

SEQ ID NO: 101 - DNA, 42 bp, Artificial Sequence
  source: /note="Description of Artificial Sequence: Synthetic primer"
cagacgtgtgctcttccgatctgattcctctccaaacccatg

SEQ ID NO: 102 - DNA, 20 bp, Artificial Sequence
  source: /note="Description of Artificial Sequence: Synthetic primer"
tgttttggggaaagttggag

SEQ ID NO: 103 - DNA, 42 bp, Artificial Sequence
  source: /note="Description of Artificial Sequence: Synthetic primer"
cagacgtgtgctcttccgatctctgtttgcccagtgtttgtg

SEQ ID NO: 104 - DNA, 20 bp, Artificial Sequence
  source: /note="Description of Artificial Sequence: Synthetic primer"
tgcaacccaactgtgtgtta

SEQ ID NO: 105 - DNA, 44 bp, Artificial Sequence
  source: /note="Description of Artificial Sequence: Synthetic primer"
cagacgtgtgctcttccgatcttttcaccaactgttctctgagc

SEQ ID NO: 106 - DNA, 20 bp, Artificial Sequence
  source: /note="Description of Artificial Sequence: Synthetic primer"
gccctgagcaacaatagcag

SEQ ID NO: 107 - DNA, 42 bp, Artificial Sequence
  source: /note="Description of Artificial Sequence: Synthetic primer"
cagacgtgtgctcttccgatctttcagctcttcactccagca

SEQ ID NO: 108 - DNA, 20 bp, Artificial Sequence
  source: /note="Description of Artificial Sequence: Synthetic primer"
aggaaaagatgtggctcacg

SEQ ID NO: 109 - DNA, 42 bp, Artificial Sequence
  source: /note="Description of Artificial Sequence: Synthetic primer"
cagacgtgtgctcttccgatctggagttggggagaactgtca

SEQ ID NO: 110 - DNA, 20 bp, Artificial Sequence
  source: /note="Description of Artificial Sequence: Synthetic primer"
tcgaataatccagggaaacc

SEQ ID NO: 111 - DNA, 42 bp, Artificial Sequence
  source: /note="Description of Artificial Sequence: Synthetic primer"
cagacgtgtgctcttccgatctaccaaagcatcacgttgaca

SEQ ID NO: 112 - DNA, 20 bp, Artificial Sequence
  source: /note="Description of Artificial Sequence: Synthetic primer"
ggctttacaaagctggcaat

SEQ ID NO: 113 - DNA, 42 bp, Artificial Sequence
  source: /note="Description of Artificial Sequence: Synthetic primer"
cagacgtgtgctcttccgatcttatgcctcttcgattgctcc

SEQ ID NO: 114 - DNA, 20 bp, Artificial Sequence
  source: /note="Description of Artificial Sequence: Synthetic primer"
ccttgagtgtgtctgcgtgt

SEQ ID NO: 115 - DNA, 42 bp, Artificial Sequence
  source: /note="Description of Artificial Sequence: Synthetic primer"
cagacgtgtgctcttccgatctccacagaattgggttccaag

SEQ ID NO: 116 - DNA, 20 bp, Artificial Sequence
  source: /note="Description of Artificial Sequence: Synthetic primer"
aactgggaaggccaggtaac

SEQ ID NO: 117 - DNA, 42 bp, Artificial Sequence
  source: /note="Description of Artificial Sequence: Synthetic primer"
cagacgtgtgctcttccgatcttgttttcaaattgccattgc

SEQ ID NO: 118 - DNA, 20 bp, Artificial Sequence
  source: /note="Description of Artificial Sequence: Synthetic primer"
ctttctccacgccatttgat

SEQ ID NO: 119 - DNA, 42 bp, Artificial Sequence
  source: /note="Description of Artificial Sequence: Synthetic primer"
cagacgtgtgctcttccgatctactaggatatggggtgggct

SEQ ID NO: 120 - DNA, 20 bp, Artificial Sequence
  source: /note="Description of Artificial Sequence: Synthetic primer"
gggatctgctcgtcatcatt

SEQ ID NO: 121 - DNA, 42 bp, Artificial Sequence
  source: /note="Description of Artificial Sequence: Synthetic primer"
cagacgtgtgctcttccgatctgtttctgcctctgagggaaa

SEQ ID NO: 122 - DNA, 20 bp, Artificial Sequence
  source: /note="Description of Artificial Sequence: Synthetic primer"
gcgtgcgcgttatttattta

SEQ ID NO: 123 - DNA, 42 bp, Artificial Sequence
  source: /note="Description of Artificial Sequence: Synthetic primer"
cagacgtgtgctcttccgatcttgtctggggaaggcaagtta

SEQ ID NO: 124 - DNA, 20 bp, Artificial Sequence
  source: /note="Description of Artificial Sequence: Synthetic primer"
gcagtcagccagaaatcaca

SEQ ID NO: 125 - DNA, 42 bp, Artificial Sequence
  source: /note="Description of Artificial Sequence: Synthetic primer"
cagacgtgtgctcttccgatctttttctcctctctgggacca

SEQ ID NO: 126 - DNA, 21 bp, Artificial Sequence
  source: /note="Description of Artificial Sequence: Synthetic primer"
tgaaaagtctccctttccaga

SEQ ID NO: 127 - DNA, 42 bp, Artificial Sequence
  source: /note="Description of Artificial Sequence: Synthetic primer"
cagacgtgtgctcttccgatctccttcagacagattccaggc

SEQ ID NO: 128 - DNA, 20 bp, Artificial Sequence
  source: /note="Description of Artificial Sequence: Synthetic primer"
ggagaggagagatggggatt

SEQ ID NO: 129 - DNA, 42 bp, Artificial Sequence
  source: /note="Description of Artificial Sequence: Synthetic primer"
cagacgtgtgctcttccgatctgagtgagtgccccttttctt

SEQ ID NO: 130 - DNA, 20 bp, Artificial Sequence
  source: /note="Description of Artificial Sequence: Synthetic primer"
ctcatgccaacaagaacctg

SEQ ID NO: 131 - DNA, 42 bp, Artificial Sequence
  source: /note="Description of Artificial Sequence: Synthetic primer"
cagacgtgtgctcttccgatcttgacccacacctgacacttc

SEQ ID NO: 132 - DNA, 19 bp, Artificial Sequence
  source: /note="Description of Artificial Sequence: Synthetic primer"
tcgtggaacacaggcaaac

SEQ ID NO: 133 - DNA, 42 bp, Artificial Sequence
  source: /note="Description of Artificial Sequence: Synthetic primer"
cagacgtgtgctcttccgatctttgcatttgtactggcaagg

SEQ ID NO: 134 - DNA, 20 bp, Artificial Sequence
  source: /note="Description of Artificial Sequence: Synthetic primer"
tcaaggcaaccagaggaaac

SEQ ID NO: 135 - DNA, 42 bp, Artificial Sequence
  source: /note="Description of Artificial Sequence: Synthetic primer"
cagacgtgtgctcttccgatctactaagggatggggcagtct

SEQ ID NO: 136 - DNA, 20 bp, Artificial Sequence
  source: /note="Description of Artificial Sequence: Synthetic primer"
accttttcgttggcatgtgt

SEQ ID NO: 137 - DNA, 42 bp, Artificial Sequence
  source: /note="Description of Artificial Sequence: Synthetic primer"
cagacgtgtgctcttccgatcttcagggaaaggactcacctg

SEQ ID NO: 138 - DNA, 20 bp, Artificial Sequence
  source: /note="Description of Artificial Sequence: Synthetic primer"
atgctgaaggcatttcttgg

SEQ ID NO: 139 - DNA, 42 bp, Artificial Sequence
  source: /note="Description of Artificial Sequence: Synthetic primer"
cagacgtgtgctcttccgatctctgtgagcatggtgcttcat

SEQ ID NO: 140 - DNA, 20 bp, Artificial Sequence
  source: /note="Description of Artificial Sequence: Synthetic primer"
gaggggagtggtgggtttat

SEQ ID NO: 141 - DNA, 42 bp, Artificial Sequence
  source: /note="Description of Artificial Sequence: Synthetic primer"
cagacgtgtgctcttccgatctcaaaagggaaagggaggatt

SEQ ID NO: 142 - DNA, 20 bp, Artificial Sequence
  source: /note="Description of Artificial Sequence: Synthetic primer"
aggggaaaactcatgagcag

SEQ ID NO: 143 - DNA, 42 bp, Artificial Sequence
  source: /note="Description of Artificial Sequence: Synthetic primer"
cagacgtgtgctcttccgatcttcactgtgcctggaccatag

SEQ ID NO: 144 - DNA, 20 bp, Artificial Sequence
  source: /note="Description of Artificial Sequence: Synthetic primer"
ttgggcagaaagaaaaatgg

SEQ ID NO: 145 - DNA, 44 bp, Artificial Sequence
  source: /note="Description of Artificial Sequence: Synthetic primer"
cagacgtgtgctcttccgatctcaaaagattccaccagactgaa

SEQ ID NO: 146 - DNA, 20 bp, Artificial Sequence
  source: /note="Description of Artificial Sequence: Synthetic primer"
cctcccccagtctctcttct

SEQ ID NO: 147 - DNA, 42 bp, Artificial Sequence
  source: /note="Description of Artificial Sequence: Synthetic primer"
cagacgtgtgctcttccgatctgagtcaggccgttgctagtc

SEQ ID NO: 148 - DNA, 20 bp, Artificial Sequence
  source: /note="Description of Artificial Sequence: Synthetic primer"
ggctgatcttcccacaacac

SEQ ID NO: 149 - DNA, 42 bp, Artificial Sequence
  source: /note="Description of Artificial Sequence: Synthetic primer"
cagacgtgtgctcttccgatctacgagggcaaagatgctaaa

SEQ ID NO: 150 - DNA, 20 bp, Artificial Sequence
  source: /note="Description of Artificial Sequence: Synthetic primer"
attcccgtgttgcttcaaac

SEQ ID NO: 151 - DNA, 42 bp, Artificial Sequence
  source: /note="Description of Artificial Sequence: Synthetic primer"
cagacgtgtgctcttccgatctagaactgccagcaggtagga

SEQ ID NO: 152 - DNA, 20 bp, Artificial Sequence
  source: /note="Description of Artificial Sequence: Synthetic primer"
cacttccctgggacattctc

SEQ ID NO: 153 - DNA, 42 bp, Artificial Sequence
  source: /note="Description of Artificial Sequence: Synthetic primer"
cagacgtgtgctcttccgatctctcactcttctccaggccag

SEQ ID NO: 154 - DNA, 20 bp, Artificial Sequence
  source: /note="Description of Artificial Sequence: Synthetic primer"
tgatgtctgtctggctgagg

SEQ ID NO: 155 - DNA, 42 bp, Artificial Sequence
  source: /note="Description of Artificial Sequence: Synthetic primer"
cagacgtgtgctcttccgatctccacacacagaggaagagca

SEQ ID NO: 156 - DNA, 20 bp, Artificial Sequence
  source: /note="Description of Artificial Sequence: Synthetic primer"
ccagcctgtaggaaaccaaa

SEQ ID NO: 157 - DNA, 42 bp, Artificial Sequence
  source: /note="Description of Artificial Sequence: Synthetic primer"
cagacgtgtgctcttccgatctctccttctatctccagggcc

SEQ ID NO: 158 - DNA, 20 bp, Artificial Sequence
  source: /note="Description of Artificial Sequence: Synthetic primer"
ggatgcaggtggtttttgat

SEQ ID NO: 159 - DNA, 47 bp, Artificial Sequence
  source: /note="Description of Artificial Sequence: Synthetic primer"
cagacgtgtgctcttccgatctcattgtacccattttacattttctt

SEQ ID NO: 160 - DNA, 22 bp, Artificial Sequence
  source: /note="Description of Artificial Sequence: Synthetic primer"
caaaccttaaacacccagaagc

SEQ ID NO: 161 - DNA, 42 bp, Artificial Sequence
  source: /note="Description of Artificial Sequence: Synthetic primer"
cagacgtgtgctcttccgatctataacaattcggcagttggc

SEQ ID NO: 162 - DNA, 20 bp, Artificial Sequence
  source: /note="Description of Artificial Sequence: Synthetic primer"
gaaccagtttcctcctgtgc

SEQ ID NO: 163 - DNA, 42 bp, Artificial Sequence
  source: /note="Description of Artificial Sequence: Synthetic primer"
cagacgtgtgctcttccgatctaagatgtggaggctgttgct

SEQ ID NO: 164 - DNA, 20 bp, Artificial Sequence
  source: /note="Description of Artificial Sequence: Synthetic primer"
gactgcggatctctgtgtca

SEQ ID NO: 165 - DNA, 42 bp, Artificial Sequence
  source: /note="Description of Artificial Sequence: Synthetic primer"
cagacgtgtgctcttccgatcttctgcactattcctttgccc

SEQ ID NO: 166 - DNA, 23 bp, Artificial Sequence
  source: /note="Description of Artificial Sequence: Synthetic primer"
tcagtatgatcttgtgctgtgct

SEQ ID NO: 167 - DNA, 42 bp, Artificial Sequence
  source: /note="Description of Artificial Sequence: Synthetic primer"
cagacgtgtgctcttccgatcttacccatgaagattggtggg

SEQ ID NO: 168 - DNA, 20 bp, Artificial Sequence
  source: /note="Description of Artificial Sequence: Synthetic primer"
cacagcatgagaggctctgt

SEQ ID NO: 169 - DNA, 42 bp, Artificial Sequence
  source: /note="Description of Artificial Sequence: Synthetic primer"
cagacgtgtgctcttccgatcttctcagttccgatttcccag

SEQ ID NO: 170 - DNA, 20 bp, Artificial Sequence
  source: /note="Description of Artificial Sequence: Synthetic primer"
tcaggatctgaggtcccaac

SEQ ID NO: 171 - DNA, 42 bp, Artificial Sequence
  source: /note="Description of Artificial Sequence: Synthetic primer"
cagacgtgtgctcttccgatcttcacctgtgtatctcacgca

SEQ ID NO: 172 - DNA, 20 bp, Artificial Sequence
  source: /note="Description of Artificial Sequence: Synthetic primer"
agagctgtctagcccaggtg

SEQ ID NO: 173 - DNA, 42 bp, Artificial Sequence
  source: /note="Description of Artificial Sequence: Synthetic primer"
cagacgtgtgctcttccgatcttggtgtcctttctctgctcc

SEQ ID NO: 174 - DNA, 20 bp, Artificial Sequence
  source: /note="Description of Artificial Sequence: Synthetic primer"
cttaacgtgggagtggaacc

SEQ ID NO: 175 - DNA, 42 bp, Artificial Sequence
  source: /note="Description of Artificial Sequence: Synthetic primer"
cagacgtgtgctcttccgatctgtgtgcaaatggcagctaga

SEQ ID NO: 176 - DNA, 20 bp, Artificial Sequence
  source: /note="Description of Artificial Sequence: Synthetic primer"
tctcagcttccaccaaggtt

SEQ ID NO: 177 - DNA, 42 bp, Artificial Sequence
  source: /note="Description of Artificial Sequence: Synthetic primer"
cagacgtgtgctcttccgatcttcactgggacacttttgcct

SEQ ID NO: 178 - DNA, 20 bp, Artificial Sequence
  source: /note="Description of Artificial Sequence: Synthetic primer"
caggggagagtgtggtgttt

SEQ ID NO: 179 - DNA, 42 bp, Artificial Sequence
  source: /note="Description of Artificial Sequence: Synthetic primer"
cagacgtgtgctcttccgatctgacatgcactcagctcttgg

SEQ ID NO: 180 - DNA, 23 bp, Artificial Sequence
  source: /note="Description of Artificial Sequence: Synthetic primer"
tgcatagttcccatgttaaatcc

SEQ ID NO: 181 - DNA, 42 bp, Artificial Sequence
  source: /note="Description of Artificial Sequence: Synthetic primer"
cagacgtgtgctcttccgatcttaccaggaatggatgtcgct

SEQ ID NO: 182 - DNA, 20 bp, Artificial Sequence
  source: /note="Description of Artificial Sequence: Synthetic primer"
acatcctacggtcccaaggt

SEQ ID NO: 183 - DNA, 41 bp, Artificial Sequence
  source: /note="Description of Artificial Sequence: Synthetic primer"
cagacgtgtgctcttccgatctgcagaagtgcaggcaccta

SEQ ID NO: 184 - DNA, 20 bp, Artificial Sequence
  source: /note="Description of Artificial Sequence: Synthetic primer"
tgcatgatcaaatgcaacct

SEQ ID NO: 185 - DNA, 43 bp, Artificial Sequence
  source: /note="Description of Artificial Sequence: Synthetic primer"
cagacgtgtgctcttccgatctttggactttgggcataaaaga

SEQ ID NO: 186 - DNA, 20 bp, Artificial Sequence
  source: /note="Description of Artificial Sequence: Synthetic primer"
aaatcacggcagttttcagc

SEQ ID NO: 187 - DNA, 42 bp, Artificial Sequence
  source: /note="Description of Artificial Sequence: Synthetic primer"
cagacgtgtgctcttccgatctctcatctgtgcactctcccc

SEQ ID NO: 188 - DNA, 20 bp, Artificial Sequence
  source: /note="Description of Artificial Sequence: Synthetic primer"
gtgggaagagaagctgatgc

SEQ ID NO: 189 - DNA, 42 bp, Artificial Sequence
  source: /note="Description of Artificial Sequence: Synthetic primer"
cagacgtgtgctcttccgatcttcaagcattatccacgtcca

SEQ ID NO: 190 - DNA, 21 bp, Artificial Sequence
  source: /note="Description of Artificial Sequence: Synthetic primer"
tgtgatgccatatcaagtcca

SEQ ID NO: 191 - DNA, 45 bp, Artificial Sequence
  source: /note="Description of Artificial Sequence: Synthetic primer"
cagacgtgtgctcttccgatcttcagtgtatgcgaaaaggttttt

SEQ ID NO: 192 - DNA, 20 bp, Artificial Sequence
  source: /note="Description of Artificial Sequence: Synthetic primer"
agcctctcttgggctttctt

SEQ ID NO: 193 - DNA, 42 bp, Artificial Sequence
  source: /note="Description of Artificial Sequence: Synthetic primer"
cagacgtgtgctcttccgatctgttttccctgcctggaactt

SEQ ID NO: 194 - DNA, 20 bp, Artificial Sequence
  source: /note="Description of Artificial Sequence: Synthetic primer"
ctttgctgctgaaggctcat

SEQ ID NO: 195 - DNA, 42 bp, Artificial Sequence
  source: /note="Description of Artificial Sequence: Synthetic primer"
cagacgtgtgctcttccgatctacaagtggtggtaaccctgg

SEQ ID NO: 196 - DNA, 20 bp, Artificial Sequence
  source: /note="Description of Artificial Sequence: Synthetic primer"
tgcttcctaaaaagcgaggt

SEQ ID NO: 197 - DNA, 42 bp, Artificial Sequence
  source: /note="Description of Artificial Sequence: Synthetic primer"
cagacgtgtgctcttccgatctgaactagggagggggaaaga

SEQ ID NO: 198 - DNA, 20 bp, Artificial Sequence
  source: /note="Description of Artificial Sequence: Synthetic primer"
gcagccaacctaagcaagat

SEQ ID NO: 199 - DNA, 42 bp, Artificial Sequence
  source: /note="Description of Artificial Sequence: Synthetic primer"
cagacgtgtgctcttccgatctatccagttactgccggtttg

SEQ ID NO: 200 - DNA, 20 bp, Artificial Sequence
  source: /note="Description of Artificial Sequence: Synthetic primer"
gaatgctgcaggacttgaga

SEQ ID NO: 201 - DNA, 42 bp, Artificial Sequence
  source: /note="Description of Artificial Sequence: Synthetic primer"
cagacgtgtgctcttccgatctacttccttgagacacggagc

SEQ ID NO: 202 - DNA, 20 bp, Artificial Sequence
  source: /note="Description of Artificial Sequence: Synthetic primer"
acccagggacttaatcagca

SEQ ID NO: 203 - DNA, 43 bp, Artificial Sequence
  source: /note="Description of Artificial Sequence: Synthetic primer"
cagacgtgtgctcttccgatctgctgatgagacagcaaccatt

SEQ ID NO: 204 - DNA, 19 bp, Artificial Sequence
  source: /note="Description of Artificial Sequence: Synthetic primer"
gacatctttgctgcctcca

SEQ ID NO: 205 - DNA, 42 bp, Artificial Sequence
  source: /note="Description of Artificial Sequence: Synthetic primer"
cagacgtgtgctcttccgatctatgagaaggacactcgctgc

SEQ ID NO: 206 - DNA, 21 bp, Artificial Sequence
  source: /note="Description of Artificial Sequence: Synthetic primer"
ttaaggagttcctgcagtcca

SEQ ID NO: 207 - DNA, 42 bp, Artificial Sequence
  source: /note="Description of Artificial Sequence: Synthetic primer"
cagacgtgtgctcttccgatcttccactgggcacagaactta

SEQ ID NO: 208 - DNA, 20 bp, Artificial Sequence
  source: /note="Description of Artificial Sequence: Synthetic primer"
tccttcgctttgcttgtctt

SEQ ID NO: 209 - DNA, 45 bp, Artificial Sequence
  source: /note="Description of Artificial Sequence: Synthetic primer"
cagacgtgtgctcttccgatctaggtggaaaaatagatgccagtc

SEQ ID NO: 210 - DNA, 19 bp, Artificial Sequence
  source: /note="Description of Artificial Sequence: Synthetic primer"
cccggaagtctatgcgttt

SEQ ID NO: 211 - DNA, 41 bp, Artificial Sequence
  source: /note="Description of Artificial Sequence: Synthetic primer"
cagacgtgtgctcttccgatctaggacatctcggtgcagtg

SEQ ID NO: 212 - DNA, 20 bp, Artificial Sequence
  source: /note="Description of Artificial Sequence: Synthetic primer"
tgtgtgaggtgtctggcttc

SEQ ID NO: 213 - DNA, 40 bp, Artificial Sequence
  source: /note="Description of Artificial Sequence: Synthetic primer"
cagacgtgtgctcttccgatctaggagcaccacgttctgg

SEQ ID NO: 214 - DNA, 20 bp, Artificial Sequence
  source: /note="Description of Artificial Sequence: Synthetic primer"
cccggagaagtatgtgacca

SEQ ID NO: 215 - DNA, 41 bp, Artificial Sequence
  source: /note="Description of Artificial Sequence: Synthetic primer"
cagacgtgtgctcttccgatctgtacttcgcccacagcatc

SEQ ID NO: 216 - DNA, 18 bp, Artificial Sequence
  source: /note="Description of Artificial Sequence: Synthetic primer"
ctgaacgagctggtgacg

SEQ ID NO: 217 - DNA, 42 bp, Artificial Sequence
  source: /note="Description of Artificial Sequence: Synthetic primer"
cagacgtgtgctcttccgatctagtacctgacttgggcatcc

SEQ ID NO: 218 - DNA, 18 bp, Artificial Sequence
  source: /note="Description of Artificial Sequence: Synthetic primer"
caagggcccatcggtctt

SEQ ID NO: 219 - DNA, 44 bp, Artificial Sequence
  source: /note="Description of Artificial Sequence: Synthetic primer"
cagacgtgtgctcttccgatctttgtgacaaaactcacacatgc

SEQ ID NO: 220 - DNA, 18 bp, Artificial Sequence
  source: /note="Description of Artificial Sequence: Synthetic primer"
caagggcccatcggtctt

SEQ ID NO: 221 - DNA, 41 bp, Artificial Sequence
  source: /note="Description of Artificial Sequence: Synthetic primer"
cagacgtgtgctcttccgatctcaaatatggtcccccatgc

SEQ ID NO: 222 - DNA, 18 bp, Artificial Sequence
  source: /note="Description of Artificial Sequence: Synthetic primer"
caagggcccatcggtctt

SEQ ID NO: 223 - DNA, 42 bp, Artificial Sequence
  source: /note="Description of Artificial Sequence: Synthetic primer"
cagacgtgtgctcttccgatctgcaaatgttgtgtcgagtgc

SEQ ID NO: 224 - DNA, 18 bp, Artificial Sequence
  source: /note="Description of Artificial Sequence: Synthetic primer"
caagggcccatcggtctt

SEQ ID NO: 225 - DNA, 42 bp, Artificial Sequence
  source: /note="Description of Artificial Sequence: Synthetic primer"
cagacgtgtgctcttccgatctaccccacttggtgacacaac

SEQ ID NO: 226 - DNA, 20 bp, Artificial Sequence
  source: /note="Description of Artificial Sequence: Synthetic primer"
ccattccgcagtactccatt

SEQ ID NO: 227 - DNA, 42 bp, Artificial Sequence
  source: /note="Description of Artificial Sequence: Synthetic primer"
cagacgtgtgctcttccgatctaaggaaaagagcaaacgtgg

SEQ ID NO: 228 - DNA, 20 bp, Artificial Sequence
  source: /note="Description of Artificial Sequence: Synthetic primer"
ttggttgacttcatggatgc

SEQ ID NO: 229 - DNA, 45 bp, Artificial Sequence
  source: /note="Description of Artificial Sequence: Synthetic primer"
cagacgtgtgctcttccgatctggaaacagcacaaatgaacttaa

SEQ ID NO: 230 - DNA, 20 bp, Artificial Sequence
  source: /note="Description of Artificial Sequence: Synthetic primer"
catcatgcagttcaacaagc

SEQ ID NO: 231 - DNA, 42 bp, Artificial Sequence
  source: /note="Description of Artificial Sequence: Synthetic primer"
cagacgtgtgctcttccgatctatgcactctgtttgcgaaga

SEQ ID NO: 232 - DNA, 20 bp, Artificial Sequence
  source: /note="Description of Artificial Sequence: Synthetic primer"
gggtgtgtttccatgtctca

SEQ ID NO: 233 - DNA, 42 bp, Artificial Sequence
  source: /note="Description of Artificial Sequence: Synthetic primer"
cagacgtgtgctcttccgatctttgaaagtgtgtgtgtccgc

SEQ ID NO: 234 - DNA, 20 bp, Artificial Sequence
  source: /note="Description of Artificial Sequence: Synthetic primer"
tcaggctgttgcatgaagaa

SEQ ID NO: 235 - DNA, 42 bp, Artificial Sequence
  source: /note="Description of Artificial Sequence: Synthetic primer"
cagacgtgtgctcttccgatctgtatgcccttgctggaccta

SEQ ID NO: 236 - DNA, 20 bp, Artificial Sequence
  source: /note="Description of Artificial Sequence: Synthetic primer"
atgcgcagtaaaaactcgtg

SEQ ID NO: 237 - DNA, 42 bp, Artificial Sequence
  source: /note="Description of Artificial Sequence: Synthetic primer"
cagacgtgtgctcttccgatcttacagttccacgctgagctg

SEQ ID NO: 238 - DNA, 21 bp, Artificial Sequence
  source: /note="Description of Artificial Sequence: Synthetic primer"
gcctgtactttcagctgggta

SEQ ID NO: 239 - DNA, 42 bp, Artificial Sequence
  source: /note="Description of Artificial Sequence: Synthetic primer"
cagacgtgtgctcttccgatctaaggtgtttgtgccatttgg

SEQ ID NO: 240 - DNA, 20 bp, Artificial Sequence
  source: /note="Description of Artificial Sequence: Synthetic primer"
ggtgagctctgattgcttca

SEQ ID NO: 241 - DNA, 42 bp, Artificial Sequence
  source: /note="Description of Artificial Sequence: Synthetic primer"
cagacgtgtgctcttccgatcttatcaggaggcagggatcac

SEQ ID NO: 242 - DNA, 19 bp, Artificial Sequence
  source: /note="Description of Artificial Sequence: Synthetic primer"
gaccgggtcagtggtctct

SEQ ID NO: 243 - DNA, 41 bp, Artificial Sequence
  source: /note="Description of Artificial Sequence: Synthetic primer"
cagacgtgtgctcttccgatctggtgatcctgagccctgac

SEQ ID NO: 244 - DNA, 20 bp, Artificial Sequence
  source: /note="Description of Artificial Sequence: Synthetic primer"
tgcagtgagctgagatcgag

SEQ ID NO: 245 - DNA, 42 bp, Artificial Sequence
  source: /note="Description of Artificial Sequence: Synthetic primer"
cagacgtgtgctcttccgatctatggaaaacatcctcatggc

SEQ ID NO: 246 - DNA, 21 bp, Artificial Sequence
  source: /note="Description of Artificial Sequence: Synthetic primer"
  source: /note="Description of Combined DNA/RNA Molecule: Synthetic primer"
cacatggccuccaaggaguaa

SEQ ID NO: 247 - DNA, 42 bp, Artificial Sequence; identical to SEQ ID NO: 25
  source: /note="Description of Artificial Sequence: Synthetic primer"

SEQ ID NO: 248 - DNA, 19 bp, Artificial Sequence
  source: /note="Description of Artificial Sequence: Synthetic primer"
gcagggtcccagtcctatg

SEQ ID NO: 249 - DNA, 42 bp, Artificial Sequence; identical to SEQ ID NO: 27
  source: /note="Description of Artificial Sequence: Synthetic primer"

SEQ ID NO: 250 - DNA, 20 bp, Artificial Sequence
  source: /note="Description of Artificial Sequence: Synthetic primer"
taggagcaggcctgagaaaa

SEQ ID NO: 251 - DNA, 42 bp, Artificial Sequence; identical to SEQ ID NO: 101
  source: /note="Description of Artificial Sequence: Synthetic primer"

SEQ ID NO: 252 - DNA, 20 bp, Artificial Sequence
  source: /note="Description of Artificial Sequence: Synthetic primer"
tccttcgctttgcttgtctt

SEQ ID NO: 253 - DNA, 45 bp, Artificial Sequence; identical to SEQ ID NO: 209
  source: /note="Description of Artificial Sequence: Synthetic primer"

SEQ ID NO: 254 - DNA, 19 bp, Artificial Sequence
  source: /note="Description of Artificial Sequence: Synthetic primer"
ggtaaacacgcctgcaaac

SEQ ID NO: 255 - DNA, 42 bp, Artificial Sequence; identical to SEQ ID NO: 69
  source: /note="Description of Artificial Sequence: Synthetic primer"

SEQ ID NO: 256 - DNA, 24 bp, Artificial Sequence
  source: /note="Description of Artificial Sequence: Synthetic primer"
caacaaagcacagtgttaaatgaa

SEQ ID NO: 257 - DNA, 42 bp, Artificial Sequence; identical to SEQ ID NO: 71
  source: /note="Description of Artificial Sequence: Synthetic primer"

SEQ ID NO: 258 - DNA, 20 bp, Artificial Sequence
  source: /note="Description of Artificial Sequence: Synthetic primer"
tgtgtgaggtgtctggcttc

SEQ ID NO: 259 - DNA, 40 bp, Artificial Sequence; identical to SEQ ID NO: 213
  source: /note="Description of Artificial Sequence: Synthetic primer"

SEQ ID NO: 260 - DNA, 20 bp, Artificial Sequence
  source: /note="Description of Artificial Sequence: Synthetic primer"
cccggagaagtatgtgacca

SEQ ID NO: 261 - DNA, 41 bp, Artificial Sequence; identical to SEQ ID NO: 215
  source: /note="Description of Artificial Sequence: Synthetic primer"

SEQ ID NO: 262 - DNA, 20 bp, Artificial Sequence
  source: /note="Description of Artificial Sequence: Synthetic primer"
tccaggaggattaccgaaaa

SEQ ID NO: 263 - DNA, 42 bp, Artificial Sequence; identical to SEQ ID NO: 29
  source: /note="Description of Artificial Sequence: Synthetic primer"

SEQ ID NO: 264 - DNA, 20 bp, Artificial Sequence
  source: /note="Description of Artificial Sequence: Synthetic primer"
agatctgagccagtcgctgt

SEQ ID NO: 265 - DNA, 43 bp, Artificial Sequence; identical to SEQ ID NO: 33
  source: /note="Description of Artificial Sequence: Synthetic primer"

SEQ ID NO: 266 - DNA, 20 bp, Artificial Sequence
  source: /note="Description of Artificial Sequence: Synthetic primer"
aaaagtgggcttgattctgc

SEQ ID NO: 267 - DNA, 42 bp, Artificial Sequence; identical to SEQ ID NO: 35
  source: /note="Description of Artificial Sequence: Synthetic primer"

SEQ ID NO: 268 - DNA, 20 bp, Artificial Sequence
  source: /note="Description of Artificial Sequence: Synthetic primer"
tgagcagatccacaggaaaa

SEQ ID NO: 269 - DNA, 44 bp, Artificial Sequence; identical to SEQ ID NO: 73
  source: /note="Description of Artificial Sequence: Synthetic primer"

SEQ ID NO: 270 - DNA, 20 bp, Artificial Sequence
  source: /note="Description of Artificial Sequence: Synthetic primer"
cccccgaaaatgttcaataa

SEQ ID NO: 271 - DNA, 41 bp, Artificial Sequence; identical to SEQ ID NO: 39
  source: /note="Description of Artificial Sequence: Synthetic primer"

SEQ ID NO: 272 - DNA, 20 bp, Artificial Sequence
  source: /note="Description of Artificial Sequence: Synthetic primer"
atattcctttgggcctctgc

SEQ ID NO: 273 - DNA, 42 bp, Artificial Sequence; identical to SEQ ID NO: 37
  source: /note="Description of Artificial Sequence: Synthetic primer"

SEQ ID NO: 274 - DNA, 20 bp, Artificial Sequence
  source: /note="Description of Artificial Sequence: Synthetic primer"
ccccaaccacttcattcttg

SEQ ID NO: 275 - DNA, 43 bp, Artificial Sequence; identical to SEQ ID NO: 51
  source: /note="Description of Artificial Sequence: Synthetic primer"

SEQ ID NO: 276 - DNA, 20 bp, Artificial Sequence
  source: /note="Description of Artificial Sequence: Synthetic primer"
aatggcaaaggaaggtggat

SEQ ID NO: 277 - DNA, 42 bp, Artificial Sequence; identical to SEQ ID NO: 31
  source: /note="Description of Artificial Sequence: Synthetic primer"

SEQ ID NO: 278 - DNA, 23 bp, Artificial Sequence
  source: /note="Description of Artificial Sequence: Synthetic primer"
tgcatagttcccatgttaaatcc

SEQ ID NO: 279 - DNA, 42 bp, Artificial Sequence; identical to SEQ ID NO: 181
  source: /note="Description of Artificial Sequence: Synthetic primer"

SEQ ID NO: 280 - DNA, 23 bp, Artificial Sequence
  source: /note="Description of Artificial Sequence: Synthetic primer"
aaatctgcagaaggaaaaatgtg

SEQ ID NO: 281 - DNA, 42 bp, Artificial Sequence; identical to SEQ ID NO: 81
  source: /note="Description of Artificial Sequence: Synthetic primer"

SEQ ID NO: 282 - DNA, 20 bp, Artificial Sequence
  source: /note="Description of Artificial Sequence: Synthetic primer"
tcgaataatccagggaaacc

SEQ ID NO: 283 - DNA, 42 bp, Artificial Sequence; identical to SEQ ID NO: 111
  source: /note="Description of Artificial Sequence: Synthetic primer"

SEQ ID NO: 284 - DNA, 20 bp, Artificial Sequence
  source: /note="Description of Artificial Sequence: Synthetic primer"
ctggctctccccaatatcct

SEQ ID NO: 285 - DNA, 42 bp, Artificial Sequence; identical to SEQ ID NO: 43
  source: /note="Description of Artificial Sequence: Synthetic primer"

SEQ ID NO: 286 - DNA, 20 bp, Artificial Sequence
  source: /note="Description of Artificial Sequence: Synthetic primer"
gcagccaacctaagcaagat

SEQ ID NO: 287 - DNA, 42 bp, Artificial Sequence; identical to SEQ ID NO: 199
  source: /note="Description of Artificial Sequence: Synthetic primer"

SEQ ID NO: 288 - DNA, 20 bp, Artificial Sequence
  source: /note="Description of Artificial Sequence: Synthetic primer"
tgcctagaggtgctcattca

SEQ ID NO: 289 - DNA, 42 bp, Artificial Sequence; identical to SEQ ID NO: 53
  source: /note="Description of Artificial Sequence: Synthetic primer"

SEQ ID NO: 290 - DNA, 19 bp, Artificial Sequence
  source: /note="Description of Artificial Sequence: Synthetic primer"
gacatctttgctgcctcca

SEQ ID NO: 291 - DNA, 42 bp, Artificial Sequence; identical to SEQ ID NO: 205
  source: /note="Description of Artificial Sequence: Synthetic primer"

SEQ ID NO: 292 - DNA, 20 bp, Artificial Sequence
  source: /note="Description of Artificial Sequence: Synthetic primer"
ttggacatagcccaagaaca

SEQ ID NO: 293 - DNA, 42 bp, Artificial Sequence; identical to SEQ ID NO: 65
  source: /note="Description of Artificial Sequence: Synthetic primer"

SEQ ID NO: 294 - DNA, 20 bp, Artificial Sequence
  source: /note="Description of Artificial Sequence: Synthetic primer"
aaatcacggcagttttcagc

SEQ ID NO: 295 - DNA, 42 bp, Artificial Sequence; identical to SEQ ID NO: 187
  source: /note="Description of Artificial Sequence: Synthetic primer"

SEQ ID NO: 296 - DNA, 20 bp, Artificial Sequence
  source: /note="Description of Artificial Sequence: Synthetic primer"
atgctgaaggcatttcttgg

SEQ ID NO: 297 - DNA, 42 bp, Artificial Sequence; identical to SEQ ID NO: 139
  source: /note="Description of Artificial Sequence: Synthetic primer"

SEQ ID NO: 298 - DNA, 20 bp, Artificial Sequence
  source: /note="Description of Artificial Sequence: Synthetic primer"
gactgcggatctctgtgtca

SEQ ID NO: 299 - DNA, 42 bp, Artificial Sequence; identical to SEQ ID NO: 165
  source: /note="Description of Artificial Sequence: Synthetic primer"

SEQ ID NO: 300 - DNA, 20 bp, Artificial Sequence
  source: /note="Description of Artificial Sequence: Synthetic primer"
ccgtgaggatgtcactcaga

SEQ ID NO: 301 - DNA, 42 bp, Artificial Sequence; identical to SEQ ID NO: 95
  source: /note="Description of Artificial Sequence: Synthetic primer"

SEQ ID NO: 302 - DNA, 20 bp, Artificial Sequence
  source: /note="Description of Artificial Sequence: Synthetic primer"
agacaggtccttttcgatgg

SEQ ID NO: 303 - DNA, 42 bp, Artificial Sequence; identical to SEQ ID NO: 47
  source: /note="Description of Artificial Sequence: Synthetic primer"

SEQ ID NO: 304 - DNA, 20 bp, Artificial Sequence
  source: /note="Description of Artificial Sequence: Synthetic primer"
tgttttggggaaagttggag

SEQ ID NO: 305 - DNA, 42 bp, Artificial Sequence; identical to SEQ ID NO: 103
  source: /note="Description of Artificial Sequence: Synthetic primer"

SEQ ID NO: 306 - DNA, 20 bp, Artificial Sequence
  source: /note="Description of Artificial Sequence: Synthetic primer"
acatcctacggtcccaaggt

SEQ ID NO: 307 - DNA, 41 bp, Artificial Sequence; identical to SEQ ID NO: 183
  source: /note="Description of Artificial Sequence: Synthetic primer"

SEQ ID NO: 308 - DNA, 20 bp, Artificial Sequence
  source: /note="Description of Artificial Sequence: Synthetic primer"
agagctgtctagcccaggtg

SEQ ID NO: 309 - DNA, 42 bp, Artificial Sequence; identical to SEQ ID NO: 173
  source: /note="Description of Artificial Sequence: Synthetic primer"

SEQ ID NO: 310 - DNA, 20 bp, Artificial Sequence
  source: /note="Description of Artificial Sequence: Synthetic primer"
tgacgtgtgttgcttttgtg

SEQ ID NO: 311 - DNA, 42 bp, Artificial Sequence
  source: /note="Description of Artificial Sequence: Synthetic primer"
cagacgtgtgctcttccgatctacttgggagaaaacaggggt

SEQ ID NO: 312 - DNA, 20 bp, Artificial Sequence
  source: /note="Description of Artificial Sequence: Synthetic primer"
gctttccactcccagctatg

SEQ ID NO: 313 - DNA, 42 bp, Artificial Sequence
  source: /note="Description of Artificial Sequence: Synthetic primer"
cagacgtgtgctcttccgatcttgctttgagtgctacggaga

SEQ ID NO: 314 - DNA, 20 bp, Artificial Sequence
  source: /note="Description of Artificial Sequence: Synthetic primer"
gggggagggatgtgaagtta

SEQ ID NO: 315 - DNA, 42 bp, Artificial Sequence
  source: /note="Description of Artificial Sequence: Synthetic primer"
cagacgtgtgctcttccgatctatcttgtctgtgattccggg

SEQ ID NO: 316 - DNA, 21 bp, Artificial Sequence
  source: /note="Description of Artificial Sequence: Synthetic primer"
acagatgacccaatgcaattc

SEQ ID NO: 317 - DNA, 42 bp, Artificial Sequence
  source: /note="Description of Artificial Sequence: Synthetic primer"
cagacgtgtgctcttccgatctgagcacctgtgatatgtgcg

SEQ ID NO: 318 - DNA, 20 bp, Artificial Sequence
  source: /note="Description of Artificial Sequence: Synthetic primer"
agaccgatgcacagtcttcc

SEQ ID NO: 319 - DNA, 42 bp, Artificial Sequence
  source: /note="Description of Artificial Sequence: Synthetic primer"
cagacgtgtgctcttccgatctcttcacgtctggcctcagtc

SEQ ID NO: 320 - DNA, 20 bp, Artificial Sequence
  source: /note="Description of Artificial Sequence: Synthetic primer"
ggagcactcaagtgtgacga

SEQ ID NO: 321 - DNA, 42 bp, Artificial Sequence
  source: /note="Description of Artificial Sequence: Synthetic primer"
cagacgtgtgctcttccgatctttttctatggagccttccga

SEQ ID NO: 322 - DNA, 20 bp, Artificial Sequence
  source: /note="Description of Artificial Sequence: Synthetic primer"
catccaattcccaaggacag

SEQ ID NO: 323 - DNA, 42 bp, Artificial Sequence
  source: /note="Description of Artificial Sequence: Synthetic primer"
cagacgtgtgctcttccgatctggtgaaggtgccgagctata

SEQ ID NO: 324 - DNA, 20 bp, Artificial Sequence
  source: /note="Description of Artificial Sequence: Synthetic primer"
gctcttcctcaaaccacgaa

SEQ ID NO: 325 - DNA, 42 bp, Artificial Sequence
  source: /note="Description of Artificial Sequence: Synthetic primer"
cagacgtgtgctcttccgatctcacactcctttgcttagccc

SEQ ID NO: 326 - DNA, 20 bp, Artificial Sequence
  source: /note="Description of Artificial Sequence: Synthetic primer"
tcctcacaccacgaatctga

SEQ ID NO: 327 - DNA, 42 bp, Artificial Sequence
  source: /note="Description of Artificial Sequence: Synthetic primer"
cagacgtgtgctcttccgatctcactcctttgcttagcccac

SEQ ID NO: 328 - DNA, 20 bp, Artificial Sequence
  source: /note="Description of Artificial Sequence: Synthetic primer"
ccagctcacctgttctccag

SEQ ID NO: 329 - DNA, 41 bp, Artificial Sequence
  source: /note="Description of Artificial Sequence: Synthetic primer"
cagacgtgtgctcttccgatctgaatcccgtacctgctgct

SEQ ID NO: 330 - DNA, 20 bp, Artificial Sequence
  source: /note="Description of Artificial Sequence: Synthetic primer"
ctaaaggactgccagccaag

SEQ ID NO: 331 - DNA, 42 bp, Artificial Sequence
  source: /note="Description of Artificial Sequence: Synthetic primer"
cagacgtgtgctcttccgatctataacctgacactggacggg

SEQ ID NO: 332 - DNA, 20 bp, Artificial Sequence
  source: /note="Description of Artificial Sequence: Synthetic primer"
cacattcctgtgcattgagg

SEQ ID NO: 333 - DNA, 42 bp, Artificial Sequence
  source: /note="Description of Artificial Sequence: Synthetic primer"
cagacgtgtgctcttccgatctatactcagttcggaaggggc

SEQ ID NO: 334 - DNA, 20 bp, Artificial Sequence
  source: /note="Description of Artificial Sequence: Synthetic primer"
gaaggagggagacatgagca

SEQ ID NO: 335 - DNA, 42 bp, Artificial Sequence
  source: /note="Description of Artificial Sequence: Synthetic primer"
cagacgtgtgctcttccgatctactggtccttagccccatct

SEQ ID NO: 336 - DNA, 20 bp, Artificial Sequence
  source: /note="Description of Artificial Sequence: Synthetic primer"
tcagttggctgacttccaca

SEQ ID NO: 337 - DNA, 42 bp, Artificial Sequence
  source: /note="Description of Artificial Sequence: Synthetic primer"
cagacgtgtgctcttccgatctttagtttgggggttttgctg

SEQ ID NO: 338 - DNA, 21 bp, Artificial Sequence
  source: /note="Description of Artificial Sequence: Synthetic primer"
tcttggccagggtagtaagaa

SEQ ID NO: 339 - DNA, 42 bp, Artificial Sequence
  source: /note="Description of Artificial Sequence: Synthetic primer"
cagacgtgtgctcttccgatctgtcagttccaatgaggtggg

SEQ ID NO: 340 - DNA, 20 bp, Artificial Sequence
  source: /note="Description of Artificial Sequence: Synthetic primer"
cgtccagaccttgttcacac

SEQ ID NO: 341 - DNA, 43 bp, Artificial Sequence
  source: /note="Description of Artificial Sequence: Synthetic primer"
cagacgtgtgctcttccgatctccacaaatagtgctcgctttc

SEQ ID NO: 342 - DNA, 20 bp, Artificial Sequence
  source: /note="Description of Artificial Sequence: Synthetic primer"
tagagggccaggacatcatc

SEQ ID NO: 343 - DNA, 42 bp, Artificial Sequence
  source: /note="Description of Artificial Sequence: Synthetic primer"
cagacgtgtgctcttccgatctttgctccttttgctatgcct

SEQ ID NO: 344 - DNA, 20 bp, Artificial Sequence
  source: /note="Description of Artificial Sequence: Synthetic primer"
tgctattgaccgatgcttca

SEQ ID NO: 345 - DNA, 42 bp, Artificial Sequence
  source: /note="Description of Artificial Sequence: Synthetic primer"
cagacgtgtgctcttccgatctgcaacgggctacagctttat

SEQ ID NO: 346 - DNA, 20 bp, Artificial Sequence
  source: /note="Description of Artificial Sequence: Synthetic primer"
gctcttgttcttgccgtttt

SEQ ID NO: 347 - DNA, 42 bp, Artificial Sequence
  source: /note="Description of Artificial Sequence: Synthetic primer"
cagacgtgtgctcttccgatctgagtccctcagtggagcaag

SEQ ID NO: 348 - DNA, 22 bp, Artificial Sequence
  source: /note="Description of Artificial Sequence: Synthetic primer"
cacaagcacattcatctcttcc

SEQ ID NO: 349 - DNA, 42 bp, Artificial Sequence
  source: /note="Description of Artificial Sequence: Synthetic primer"
cagacgtgtgctcttccgatctattcagggccagcttcataa

SEQ ID NO: 350 - DNA, 20 bp, Artificial Sequence
  source: /note="Description of Artificial Sequence: Synthetic primer"
tacttcaagggagccattcc

SEQ ID NO: 351 - DNA, 42 bp, Artificial Sequence
  source: /note="Description of Artificial Sequence: Synthetic primer"
cagacgtgtgctcttccgatcttttgtaactgtgcagggcag

SEQ ID NO: 352 - DNA, 21 bp, Artificial Sequence
  source: /note="Description of Artificial Sequence: Synthetic primer"
agcaacgtggagtcagtctgt

SEQ ID NO: 353 - DNA, 42 bp, Artificial Sequence
  source: /note="Description of Artificial Sequence: Synthetic primer"
cagacgtgtgctcttccgatctctcaccttctcttgccttgg

SEQ ID NO: 354 - DNA, 21 bp, Artificial Sequence
  source: /note="Description of Artificial Sequence: Synthetic primer"
ttattttctggggctgtcaga

SEQ ID NO: 355 - DNA, 42 bp, Artificial Sequence
  source: /note="Description of Artificial Sequence: Synthetic primer"
cagacgtgtgctcttccgatctcattctggcactcaggtgaa

SEQ ID NO: 356 - DNA, 20 bp, Artificial Sequence
  source: /note="Description of Artificial Sequence: Synthetic primer"
tgatcaagcacctgagaacg

SEQ ID NO: 357 - DNA, 42 bp, Artificial Sequence
  source: /note="Description of Artificial Sequence: Synthetic primer"
cagacgtgtgctcttccgatcttaccagtgcaccatctgcac

SEQ ID NO: 358 - DNA, 21 bp, Artificial Sequence
  source: /note="Description of Artificial Sequence: Synthetic primer"
tgcaaaacccagaagctaaaa

SEQ ID NO: 359 - DNA, 42 bp, Artificial Sequence
  source: /note="Description of Artificial Sequence: Synthetic primer"
cagacgtgtgctcttccgatctgttctgtgcaaatggcattc

SEQ ID NO: 360 - DNA, 20 bp, Artificial Sequence
  source: /note="Description of Artificial Sequence: Synthetic primer"
agagctgtgtggagctggat

SEQ ID NO: 361 - DNA, 42 bp, Artificial Sequence
  source: /note="Description of Artificial Sequence: Synthetic primer"
cagacgtgtgctcttccgatctggagtcttctgctttgctgg

SEQ ID NO: 362 - DNA, 20 bp, Artificial Sequence
  source: /note="Description of Artificial Sequence: Synthetic primer"
gccctcttgccaggatattt

SEQ ID NO: 363 - DNA, 42 bp, Artificial Sequence
  source: /note="Description of Artificial Sequence: Synthetic primer"
cagacgtgtgctcttccgatctgcatgtaagttgtcccccat

SEQ ID NO: 364 - DNA, 20 bp, Artificial Sequence
  source: /note="Description of Artificial Sequence: Synthetic primer"
ctggcctctgctcaactagc

SEQ ID NO: 365 - DNA, 42 bp, Artificial Sequence
  source: /note="Description of Artificial Sequence: Synthetic primer"
cagacgtgtgctcttccgatctatggtacaagcaatgcctgc

SEQ ID NO: 366 - DNA, 20 bp, Artificial Sequence
  source: /note="Description of Artificial Sequence: Synthetic primer"
cagcctcaaggggaaggtat

SEQ ID NO: 367 - DNA, 42 bp, Artificial Sequence
  source: /note="Description of Artificial Sequence: Synthetic primer"
cagacgtgtgctcttccgatcttgcttaacccatggatcctg

SEQ ID NO: 368 - DNA, 20 bp, Artificial Sequence
  source: /note="Description of Artificial Sequence: Synthetic primer"
ccctgcagtcacagctacac

SEQ ID NO: 369 - DNA, 42 bp, Artificial Sequence
  source: /note="Description of Artificial Sequence: Synthetic primer"
cagacgtgtgctcttccgatcttcagggctggtcttttagga

SEQ ID NO: 370 - DNA, 23 bp, Artificial Sequence
  source: /note="Description of Artificial Sequence: Synthetic primer"
tgggataatgtaaaactggtgct

SEQ ID NO: 371 - DNA, 42 bp, Artificial Sequence
  source: /note="Description of Artificial Sequence: Synthetic primer"
cagacgtgtgctcttccgatctcatccccatgatatttggga

SEQ ID NO: 372 - DNA, 20 bp, Artificial Sequence
  source: /note="Description of Artificial Sequence: Synthetic primer"
agctagcctgagagggaacc

SEQ ID NO: 373 - DNA, 42 bp, Artificial Sequence
  source: /note="Description of Artificial Sequence: Synthetic primer"
cagacgtgtgctcttccgatcttcctccagaccattcaggac

SEQ ID NO: 374 - DNA, 20 bp, Artificial Sequence
  source: /note="Description of Artificial Sequence: Synthetic primer"
ggctctgccttgcactattt

SEQ ID NO: 375 - DNA, 41 bp, Artificial Sequence
  source: /note="Description of Artificial Sequence: Synthetic primer"
cagacgtgtgctcttccgatctctcttcctcccttccatgc

SEQ ID NO: 376 - DNA, 20 bp, Artificial Sequence
  source: /note="Description of Artificial Sequence: Synthetic primer"
taaggcccaaagtgggtaca

SEQ ID NO: 377 - DNA, 42 bp, Artificial Sequence
  source: /note="Description of Artificial Sequence: Synthetic primer"
cagacgtgtgctcttccgatcttaggaagcacgaggaaagga

SEQ ID NO: 378 - DNA, 20 bp, Artificial Sequence
  source: /note="Description of Artificial Sequence: Synthetic primer"
accctctctccctccctttc

SEQ ID NO: 379 - DNA, 42 bp, Artificial Sequence
  source: /note="Description of Artificial Sequence: Synthetic primer"
cagacgtgtgctcttccgatcttagttggctatgctggcatg

SEQ ID NO: 380 - DNA, 21 bp, Artificial Sequence
  source: /note="Description of Artificial Sequence: Synthetic primer"
gcctggtagaattggcttttc

SEQ ID NO: 381 - DNA, 45 bp, Artificial Sequence; identical to SEQ ID NO: 91
  source: /note="Description of Artificial Sequence: Synthetic primer"

SEQ ID NO: 382 - DNA, 20 bp, Artificial Sequence
  source: /note="Description of Artificial Sequence: Synthetic primer"
caggggagagtgtggtgttt

SEQ ID NO: 383 - DNA, 42 bp, Artificial Sequence
  source: /note="Description of Artificial Sequence: Synthetic primer"
cagacgtgtgctcttccgatctactcagctcttggctccact

SEQ ID NO: 384 - DNA, 21 bp, Artificial Sequence
  source: /note="Description of Artificial Sequence: Synthetic primer"
acatcaagctccattgtttcg

SEQ ID NO: 385 - DNA, 43 bp, Artificial Sequence
  source: /note="Description of Artificial Sequence: Synthetic primer"
cagacgtgtgctcttccgatcttttgcctgcactctttgtagg

SEQ ID NO: 386 - DNA, 20 bp, Artificial Sequence
  source: /note="Description of Artificial Sequence: Synthetic primer"
gcctggcacgtaatagcttg

SEQ ID NO: 387 - DNA, 42 bp, Artificial Sequence
  source: /note="Description of Artificial Sequence: Synthetic primer"
cagacgtgtgctcttccgatctaggaaagaaatgcccttggt

SEQ ID NO: 388 - DNA, 20 bp, Artificial Sequence
  source: /note="Description of Artificial Sequence: Synthetic primer"
gaggatgtgtggcattttca

SEQ ID NO: 389 - DNA, 42 bp, Artificial Sequence
  source: /note="Description of Artificial Sequence: Synthetic primer"
cagacgtgtgctcttccgatctggttcctaggtgagcaggtg

SEQ ID NO: 390 - DNA, 20 bp, Artificial Sequence
  source: /note="Description of Artificial Sequence: Synthetic primer"
agcaggctgtacacagcaga

SEQ ID NO: 391 - DNA, 42 bp, Artificial Sequence
  source: /note="Description of Artificial Sequence: Synthetic primer"
cagacgtgtgctcttccgatctgacactaggcacattggctg

SEQ ID NO: 392 - DNA, 20 bp, Artificial Sequence
  source: /note="Description of Artificial Sequence: Synthetic primer"
actgtgccctcatccagaac

SEQ ID NO: 393 - DNA, 42 bp, Artificial Sequence
  source: /note="Description of Artificial Sequence: Synthetic primer"
cagacgtgtgctcttccgatctaacgacgccaaggtgatact

SEQ ID NO: 394 - DNA, 21 bp, Artificial Sequence
  source: /note="Description of Artificial Sequence: Synthetic primer"
tggtgaaatgcagagtcaatg

SEQ ID NO: 395 - DNA, 42 bp, Artificial Sequence
  source: /note="Description of Artificial Sequence: Synthetic primer"
cagacgtgtgctcttccgatcttcaggaggaaggcttacacc

SEQ ID NO: 396 - DNA, 20 bp, Artificial Sequence
  source: /note="Description of Artificial Sequence: Synthetic primer"
tgaattttgcttggtggatg

SEQ ID NO: 397 - DNA, 43 bp, Artificial Sequence
  source: /note="Description of Artificial Sequence: Synthetic primer"
cagacgtgtgctcttccgatcttgtcagtggaagaagcagatg

SEQ ID NO: 398 - DNA, 20 bp, Artificial Sequence
  source: /note="Description of Artificial Sequence: Synthetic primer"
cagtgagaatgagggccaag

SEQ ID NO: 399 - DNA, 42 bp, Artificial Sequence
  source: /note="Description of Artificial Sequence: Synthetic primer"
cagacgtgtgctcttccgatctgaatgagggccaagaaagag

SEQ ID NO: 400 - DNA, 20 bp, Artificial Sequence
  source: /note="Description of Artificial Sequence: Synthetic primer"
aaaatgaaaccctccccaaa

SEQ ID NO: 401 - DNA, 42 bp, Artificial Sequence
  source: /note="Description of Artificial Sequence: Synthetic primer"
cagacgtgtgctcttccgatcttcctttggagattaaggccc

SEQ ID NO: 402 - DNA, 20 bp, Artificial Sequence
  source: /note="Description of Artificial Sequence: Synthetic primer"
ctgcatcaatgctcaaggaa

SEQ ID NO: 403 - DNA, 42 bp, Artificial Sequence
  source: /note="Description of Artificial Sequence: Synthetic primer"
cagacgtgtgctcttccgatctccaaggctgctctgtttctt

SEQ ID NO: 404 - DNA, 20 bp, Artificial Sequence
  source: /note="Description of Artificial Sequence: Synthetic primer"
aaatcaagctcccaaggtca

SEQ ID NO: 405 - DNA, 42 bp, Artificial Sequence
  source: /note="Description of Artificial Sequence: Synthetic primer"
cagacgtgtgctcttccgatcttgtgaatgacttggtccctg

SEQ ID NO: 406 - DNA, 19 bp, Artificial Sequence
  source: /note="Description of Artificial Sequence: Synthetic primer"
atgccccaaagcgattttt

SEQ ID NO: 407 - DNA, 42 bp, Artificial Sequence
  source: /note="Description of Artificial Sequence: Synthetic primer"
cagacgtgtgctcttccgatctcaaaggaaaccaatgccact

SEQ ID NO: 408 - DNA, 20 bp, Artificial Sequence
  source: /note="Description of Artificial Sequence: Synthetic primer"
tccctcattgaaagatgcaa

SEQ ID NO: 409 - DNA, 42 bp, Artificial Sequence
  source: /note="Description of Artificial Sequence: Synthetic primer"
cagacgtgtgctcttccgatcttagaatcattaggccaggcg

SEQ ID NO: 410 - DNA, 20 bp, Artificial Sequence
  source: /note="Description of Artificial Sequence: Synthetic primer"
tgcaagccatttatgggaat

SEQ ID NO: 411 - DNA, 44 bp, Artificial Sequence
  source: /note="Description of Artificial Sequence: Synthetic primer"
cagacgtgtgctcttccgatctccttgggttttcttttcaattc

SEQ ID NO: 412 - DNA, 20 bp, Artificial Sequence
  source: /note="Description of Artificial Sequence: Synthetic primer"
atttccatggtgctccagtc

SEQ ID NO: 413 - DNA, 42 bp, Artificial Sequence
  source: /note="Description of Artificial Sequence: Synthetic primer"
cagacgtgtgctcttccgatctagagaagcagaagtcgctcg

SEQ ID NO: 414 - DNA, 18 bp, Artificial Sequence
  source: /note="Description of Artificial Sequence: Synthetic primer"
ctgctggccctgtacctg

SEQ ID NO: 415 - DNA, 40 bp, Artificial Sequence
  source: /note="Description of Artificial Sequence: Synthetic primer"
cagacgtgtgctcttccgatctctccaccctggccaagat

SEQ ID NO: 416 - DNA, 21 bp, Artificial Sequence
  source: /note="Description of Artificial Sequence: Synthetic primer"
ttcagctgacttggacaacct

SEQ ID NO: 417 - DNA, 42 bp, Artificial Sequence
  source: /note="Description of Artificial Sequence: Synthetic primer"
cagacgtgtgctcttccgatctggacaacctgactggctttg

SEQ ID NO: 418 - DNA, 20 bp, Artificial Sequence
  source: /note="Description of Artificial Sequence: Synthetic primer"
gggtgttggtgaacttggtt

SEQ ID NO: 419 - DNA, 42 bp, Artificial Sequence
  source: /note="Description of Artificial Sequence: Synthetic primer"
cagacgtgtgctcttccgatcttttaatatggatgccgtggg

SEQ ID NO: 420 - DNA, 20 bp, Artificial Sequence
  source: /note="Description of Artificial Sequence: Synthetic primer"
gttgcccagtgtgtttctga

SEQ ID NO: 421 - DNA, 42 bp, Artificial Sequence
  source: /note="Description of Artificial Sequence: Synthetic primer"
cagacgtgtgctcttccgatctaaccaggcaacttgggaact

SEQ ID NO: 422 - DNA, 20 bp, Artificial Sequence
  source: /note="Description of Artificial Sequence: Synthetic primer"
ccattccgcagtactccatt

SEQ ID NO: 423 - DNA, 42 bp, Artificial Sequence; identical to SEQ ID NO: 227
  source: /note="Description of Artificial Sequence: Synthetic primer"

SEQ ID NO: 424 - DNA, 20 bp, Artificial Sequence
  source: /note="Description of Artificial Sequence: Synthetic primer"
ttggttgacttcatggatgc

SEQ ID NO: 425 - DNA, 45 bp, Artificial Sequence; identical to SEQ ID NO: 229
  source: /note="Description of Artificial Sequence: Synthetic primer"

SEQ ID NO: 426 - DNA, 20 bp, Artificial Sequence
  source: /note="Description of Artificial Sequence: Synthetic primer"
catcatgcagttcaacaagc

SEQ ID NO: 427 - DNA, 42 bp, Artificial Sequence; identical to SEQ ID NO: 231
  source: /note="Description of Artificial Sequence: Synthetic primer"

SEQ ID NO: 428 - DNA, 20 bp, Artificial Sequence
  source: /note="Description of Artificial Sequence: Synthetic primer"
gggtgtgtttccatgtctca

SEQ ID NO: 429 - DNA, 42 bp, Artificial Sequence; identical to SEQ ID NO: 233
  source: /note="Description of Artificial Sequence: Synthetic primer"

SEQ ID NO: 430 - DNA, 20 bp, Artificial Sequence
  source: /note="Description of Artificial Sequence: Synthetic primer"
tcaggctgttgcatgaagaa

SEQ ID NO: 431 - DNA, 42 bp, Artificial Sequence; identical to SEQ ID NO: 235
  source: /note="Description of Artificial Sequence: Synthetic primer"

SEQ ID NO: 432 - DNA, 20 bp, Artificial Sequence
  source: /note="Description of Artificial Sequence: Synthetic primer"
atgcgcagtaaaaactcgtg

SEQ ID NO: 433 - DNA, 42 bp, Artificial Sequence; identical to SEQ ID NO: 237
  source: /note="Description of Artificial Sequence: Synthetic primer"

SEQ ID NO: 434 - DNA, 21 bp, Artificial Sequence
  source: /note="Description of Artificial Sequence: Synthetic primer"
gcctgtactttcagctgggta

SEQ ID NO: 435 - DNA, 42 bp, Artificial Sequence; identical to SEQ ID NO: 239
  source: /note="Description of Artificial Sequence: Synthetic primer"

SEQ ID NO: 436 - DNA, 20 bp, Artificial Sequence
  source: /note="Description of Artificial Sequence: Synthetic primer"
ggtgagctctgattgcttca

SEQ ID NO: 437 - DNA, 42 bp, Artificial Sequence; identical to SEQ ID NO: 241
  source: /note="Description of Artificial Sequence: Synthetic primer"

SEQ ID NO: 438 - DNA, 19 bp, Artificial Sequence
  source: /note="Description of Artificial Sequence: Synthetic primer"
gaccgggtcagtggtctct

SEQ ID NO: 439 - DNA, 41 bp, Artificial Sequence; identical to SEQ ID NO: 243
  source: /note="Description of Artificial Sequence: Synthetic primer"

SEQ ID NO: 440 - DNA, 20 bp, Artificial Sequence
  source: /note="Description of Artificial Sequence: Synthetic primer"
tgcagtgagctgagatcgag

SEQ ID NO: 441 - DNA, 42 bp, Artificial Sequence; identical to SEQ ID NO: 245
  source: /note="Description of Artificial Sequence: Synthetic primer"

SEQ ID NO: 442 - DNA, 21 bp, Artificial Sequence
  source: /note="Description of Artificial Sequence: Synthetic primer"
  source: /note="Description of Combined DNA/RNA Molecule: Synthetic primer"
cacatggccuccaaggaguaa

SEQ ID NO: 443 - DNA, 42 bp, Artificial Sequence; identical to SEQ ID NO: 25
  source: /note="Description of Artificial Sequence: Synthetic primer"

SEQ ID NO: 444 - DNA, 20 bp, Artificial Sequence
  source: /note="Description of Artificial Sequence: Synthetic primer"
gacttcaacagcgacaccca

SEQ ID NO: 445 - DNA, 42 bp, Artificial Sequence
  source: /note="Description of Artificial Sequence: Synthetic primer"
cagacgtgtgctcttccgatctgccctcaacgaccactttgt

SEQ ID NO: 446 - DNA, 20 bp, Artificial Sequence
  source: /note="Description of Artificial Sequence: Synthetic primer"
gaaaacgcatcctggaccca

SEQ ID NO: 447 - DNA, 43 bp, Artificial Sequence
  source: /note="Description of Artificial Sequence: Synthetic primer"
cagacgtgtgctcttccgatcttgatgtcattgccactctgct

SEQ ID NO: 448 - DNA, 20 bp, Artificial Sequence
  source: /note="Description of Artificial Sequence: Synthetic primer"
aagttgtcccccatcccaaa

SEQ ID NO: 449 - DNA, 43 bp, Artificial Sequence
  source: /note="Description of Artificial Sequence: Synthetic primer"
cagacgtgtgctcttccgatctctggggatggactgggtaaat

SEQ ID NO: 450 - DNA, 20 bp, Artificial Sequence
  source: /note="Description of Artificial Sequence: Synthetic primer"
actgctgtcccaaacatgca

SEQ ID NO: 451 - DNA, 43 bp, Artificial Sequence
  source: /note="Description of Artificial Sequence: Synthetic primer"
cagacgtgtgctcttccgatctatgcctgcccattggagagaa

SEQ ID NO: 452 - DNA, 20 bp, Artificial Sequence
  source: /note="Description of Artificial Sequence: Synthetic primer"
ccaccatctttgcaggttgc

SEQ ID NO: 453 - DNA, 42 bp, Artificial Sequence
  source: /note="Description of Artificial Sequence: Synthetic primer"
cagacgtgtgctcttccgatctgctgtccagttcccagaagg

SEQ ID NO: 454 - DNA, 20 bp, Artificial Sequence
  source: /note="Description of Artificial Sequence: Synthetic primer"
ctgggagagggggtagctag

SEQ ID NO: 455 - DNA, 42 bp, Artificial Sequence
  source: /note="Description of Artificial Sequence: Synthetic primer"
cagacgtgtgctcttccgatctaccacttccctcagtcccaa

SEQ ID NO: 456 - DNA, 20 bp, Artificial Sequence
  source: /note="Description of Artificial Sequence: Synthetic primer"
acagaagcagcgtcagtacc

SEQ ID NO: 457 - DNA, 41 bp, Artificial Sequence
  source: /note="Description of Artificial Sequence: Synthetic primer"
cagacgtgtgctcttccgatctgggtctcttgagtcccgtg

SEQ ID NO: 458 - DNA, 20 bp, Artificial Sequence
  source: /note="Description of Artificial Sequence: Synthetic primer"
ggggagagtgtggtgtttcc

SEQ ID NO: 459 - DNA, 42 bp, Artificial Sequence
  source: /note="Description of Artificial Sequence: Synthetic primer"
cagacgtgtgctcttccgatctctcttggctccactgggatg

SEQ ID NO: 460 - DNA, 20 bp, Artificial Sequence
  source: /note="Description of Artificial Sequence: Synthetic primer"
atcaatggtccaagccgcat

SEQ ID NO: 461 - DNA, 42 bp, Artificial Sequence
  source: /note="Description of Artificial Sequence: Synthetic primer"
cagacgtgtgctcttccgatctaggtcacagatcttcccccg

SEQ ID NO: 462 - DNA, 20 bp, Artificial Sequence
  source: /note="Description of Artificial Sequence: Synthetic primer"
ctttccagtcctacggagcc

SEQ ID NO: 463 - DNA, 42 bp, Artificial Sequence
  source: /note="Description of Artificial Sequence: Synthetic primer"
cagacgtgtgctcttccgatcttgctctgaaccccaatcctc

SEQ ID NO: 464 - DNA, 20 bp, Artificial Sequence
  source: /note="Description of Artificial Sequence: Synthetic primer"
accatcacaggcatgttcct

SEQ ID NO: 465 - DNA, 42 bp, Artificial Sequence
  source: /note="Description of Artificial Sequence: Synthetic primer"
cagacgtgtgctcttccgatcttgtagatgacctggcttgcc

SEQ ID NO: 466 - DNA, 20 bp, Artificial Sequence
  source: /note="Description of Artificial Sequence: Synthetic primer"
gcatctcatgagtgccaagc

SEQ ID NO: 467 - DNA, 43 bp, Artificial Sequence
  source: /note="Description of Artificial Sequence: Synthetic primer"
cagacgtgtgctcttccgatctcctgcccccagaccttttatc

SEQ ID NO: 468 - DNA, 20 bp, Artificial Sequence
  source: /note="Description of Artificial Sequence: Synthetic primer"
tgcagagccttgtcgttaca

SEQ ID NO: 469 - DNA, 42 bp, Artificial Sequence
  source: /note="Description of Artificial Sequence: Synthetic primer"
cagacgtgtgctcttccgatctcgtgacagagtgccttttcg

SEQ ID NO: 470 - DNA, 21 bp, Artificial Sequence
  source: /note="Description of Artificial Sequence: Synthetic primer"
aggtgaagatgacagtgcagg

SEQ ID NO: 471 - DNA, 42 bp, Artificial Sequence
  source: /note="Description of Artificial Sequence: Synthetic primer"
cagacgtgtgctcttccgatctaggccctcttgtgtgtaaca

SEQ ID NO: 472 - DNA, 20 bp, Artificial Sequence
  source: /note="Description of Artificial Sequence: Synthetic primer"
ggaaccatgtgccaagttgc

SEQ ID NO: 473 - DNA, 42 bp, Artificial Sequence
  source: /note="Description of Artificial Sequence: Synthetic primer"
cagacgtgtgctcttccgatctcctttgttgtgcgagggtgt

SEQ ID NO: 474 - DNA, 20 bp, Artificial Sequence
  source: /note="Description of Artificial Sequence: Synthetic primer"
agtgttgctgacagtgcaga

SEQ ID NO: 475 - DNA, 43 bp, Artificial Sequence
  source: /note="Description of Artificial Sequence: Synthetic primer"
cagacgtgtgctcttccgatctccaaagaagacacagaccggt

SEQ ID NO: 476 - DNA, 20 bp, Artificial Sequence
  source: /note="Description of Artificial Sequence: Synthetic primer"
ttgccacaaagcctggaatc

SEQ ID NO: 477 - DNA, 42 bp, Artificial Sequence
  source: /note="Description of Artificial Sequence: Synthetic primer"
cagacgtgtgctcttccgatctaaagcaaccttgtcccgcct

SEQ ID NO: 478 - DNA, 20 bp, Artificial Sequence
  source: /note="Description of Artificial Sequence: Synthetic primer"
ggagtccagcgaatgacgtc

SEQ ID NO: 479 - DNA, 42 bp, Artificial Sequence
  source: /note="Description of Artificial Sequence: Synthetic primer"
cagacgtgtgctcttccgatctcatggccacgttgtcattgt

SEQ ID NO: 480 - DNA, 20 bp, Artificial Sequence
  source: /note="Description of Artificial Sequence: Synthetic primer"
caacacccaggggatcagtg

SEQ ID NO: 481 - DNA, 42 bp, Artificial Sequence
  source: /note="Description of Artificial Sequence: Synthetic primer"
cagacgtgtgctcttccgatctccaccctccacaggaaattg

SEQ ID NO: 482 - DNA, 19 bp, Artificial Sequence
  source: /note="Description of Artificial Sequence: Synthetic primer"
agctgtaccagggggagag

SEQ ID NO: 483 - DNA, 43 bp, Artificial Sequence
  source: /note="Description of Artificial Sequence: Synthetic primer"
cagacgtgtgctcttccgatctctttggagaagacagtggcga

SEQ ID NO: 484 - DNA, 21 bp, Artificial Sequence
  source: /note="Description of Artificial Sequence: Synthetic primer"
ggaagacagccagatccagtg

SEQ ID NO: 485 - DNA, 42 bp, Artificial Sequence
  source: /note="Description of Artificial Sequence: Synthetic primer"
cagacgtgtgctcttccgatctttgtgcagaccaagagcacc

SEQ ID NO: 486 - DNA, 20 bp, Artificial Sequence
  source: /note="Description of Artificial Sequence: Synthetic primer"
gggctgagaatgaggcagtt

SEQ ID NO: 487 - DNA, 42 bp, Artificial Sequence
  source: /note="Description of Artificial Sequence: Synthetic primer"
cagacgtgtgctcttccgatctggaaagcgacaagggtgaac

SEQ ID NO: 488 - DNA, 19 bp, Artificial Sequence
  source: /note="Description of Artificial Sequence: Synthetic primer"
acttaacagctgcaggggc

SEQ ID NO: 489 - DNA, 45 bp, Artificial Sequence
  source: /note="Description of Artificial Sequence: Synthetic primer"
cagacgtgtgctcttccgatctactaacttgaaccgtgtttaagg

SEQ ID NO: 490 - DNA, 20 bp, Artificial Sequence
  source: /note="Description of Artificial Sequence: Synthetic primer"
ttataaccatcagcccgcca

SEQ ID NO: 491 - DNA, 42 bp, Artificial Sequence
  source: /note="Description of Artificial Sequence: Synthetic primer"
cagacgtgtgctcttccgatctagaaaaggggctggaaaggg

SEQ ID NO: 492 - DNA, 21 bp, Artificial Sequence
  source: /note="Description of Artificial Sequence: Synthetic primer"
accaaagcatcacgttgacat

SEQ ID NO: 493 - DNA, 42 bp, Artificial Sequence
  source: /note="Description of Artificial Sequence: Synthetic primer"
cagacgtgtgctcttccgatctacatgtgaatgttgagccca

SEQ ID NO: 494 - DNA, 20 bp, Artificial Sequence
  source: /note="Description of Artificial Sequence: Synthetic primer"
ctcttcagcatcccccgtac

SEQ ID NO: 495 - DNA, 42 bp, Artificial Sequence
  source: /note="Description of Artificial Sequence: Synthetic primer"
cagacgtgtgctcttccgatctgcccccaaatgaaagcttga

SEQ ID NO: 496 - DNA, 20 bp, Artificial Sequence
  source: /note="Description of Artificial Sequence: Synthetic primer"
ggagagcgtccattccagtg

SEQ ID NO: 497 - DNA, 41 bp, Artificial Sequence
  source: /note="Description of Artificial Sequence: Synthetic primer"
cagacgtgtgctcttccgatctatccacctgaagctgcacc

SEQ ID NO: 498 - DNA, 20 bp, Artificial Sequence
  source: /note="Description of Artificial Sequence: Synthetic primer"
aatgtaccagccagtcagcg

SEQ ID NO: 499 - DNA, 42 bp, Artificial Sequence
  source: /note="Description of Artificial Sequence: Synthetic primer"
cagacgtgtgctcttccgatctggttttggtggagctgacga

SEQ ID NO: 500 - DNA, 20 bp, Artificial Sequence
  source: /note="Description of Artificial Sequence: Synthetic primer"
tttactcatcgggcagccac

SEQ ID NO: 501 - DNA, 42 bp, Artificial Sequence
  source: /note="Description of Artificial Sequence: Synthetic primer"
cagacgtgtgctcttccgatcttgtttgcccagtgtttgtgc

SEQ ID NO: 502 - DNA, 21 bp, Artificial Sequence
  source: /note="Description of Artificial Sequence: Synthetic primer"
gctgtagacaggtccttttcg

SEQ ID NO: 503 - DNA, 47 bp, Artificial Sequence
  source: /note="Description of Artificial Sequence: Synthetic primer"
cagacgtgtgctcttccgatctagtgttggaaaatgtgcaatatgtg

SEQ ID NO: 504 - DNA, 20 bp, Artificial Sequence
  source: /note="Description of Artificial Sequence: Synthetic primer"
gggtctggtgggcatcatta

SEQ ID NO: 505 - DNA, 42 bp, Artificial Sequence
  source: /note="Description of Artificial Sequence: Synthetic primer"
cagacgtgtgctcttccgatctgcctcttcgattgctccgta

SEQ ID NO: 506 - DNA, 20 bp, Artificial Sequence
  source: /note="Description of Artificial Sequence: Synthetic primer"
aggtcaatgccagagacgga

SEQ ID NO: 507 - DNA, 49 bp, Artificial Sequence
  source: /note="Description of Artificial Sequence: Synthetic primer"
cagacgtgtgctcttccgatctatcagcatacctttattgtgatctatc

SEQ ID NO: 508 - DNA, 20 bp, Artificial Sequence
  source: /note="Description of Artificial Sequence: Synthetic primer"
tggcatgtgagtcattgctc

SEQ ID NO: 509 - DNA, 42 bp, Artificial Sequence
  source: /note="Description of Artificial Sequence: Synthetic primer"
cagacgtgtgctcttccgatctttttgatgtgaggggcggat

SEQ ID NO: 510 - DNA, 20 bp, Artificial Sequence
  source: /note="Description of Artificial Sequence: Synthetic primer"
tactttttcgcctcccaggg

SEQ ID NO: 511 - DNA, 42 bp, Artificial Sequence
  source: /note="Description of Artificial Sequence: Synthetic primer"
cagacgtgtgctcttccgatcttcctgccccaccaagatcat

SEQ ID NO: 512 - DNA, 20 bp, Artificial Sequence
  source: /note="Description of Artificial Sequence: Synthetic primer"
tgccacggcctttccttaaa

SEQ ID NO: 513 - DNA, 42 bp, Artificial Sequence
  source: /note="Description of Artificial Sequence: Synthetic primer"
cagacgtgtgctcttccgatctttgtctaagtgcaaccgcct

SEQ ID NO: 514 - DNA, 20 bp, Artificial Sequence
  source: /note="Description of Artificial Sequence: Synthetic primer"
ctcctgacagaaggtgccac

SEQ ID NO: 515 - DNA, 42 bp, Artificial Sequence
  source: /note="Description of Artificial Sequence: Synthetic primer"
cagacgtgtgctcttccgatctggtgattggaccaggccatt

SEQ ID NO: 516 - DNA, 20 bp, Artificial Sequence
  source: /note="Description of Artificial Sequence: Synthetic primer"
gactggctacgtagttcggg

SEQ ID NO: 517 - DNA, 42 bp, Artificial Sequence
  source: /note="Description of Artificial Sequence: Synthetic primer"
cagacgtgtgctcttccgatcttttgcttagaaggatggcgc

SEQ ID NO: 518 - DNA, 20 bp, Artificial Sequence
  source: /note="Description of Artificial Sequence: Synthetic primer"
agctacggaactcttgtgcg

SEQ ID NO: 519 - DNA, 42 bp, Artificial Sequence
  source: /note="Description of Artificial Sequence: Synthetic primer"
cagacgtgtgctcttccgatctcaaccttggctgagtcttga

SEQ ID NO: 520 - DNA, 20 bp, Artificial Sequence
  source: /note="Description of Artificial Sequence: Synthetic primer"
tcagtctttaggggttgggc

SEQ ID NO: 521 - DNA, 45 bp, Artificial Sequence
  source: /note="Description of Artificial Sequence: Synthetic primer"
cagacgtgtgctcttccgatctatgtgcatttcaatcccacgtac

SEQ ID NO: 522 - DNA, 21 bp, Artificial Sequence
  source: /note="Description of Artificial Sequence: Synthetic primer"
ccagtctagtttctgggcagg

SEQ ID NO: 523 - DNA, 45 bp, Artificial Sequence
  source: /note="Description of Artificial Sequence: Synthetic primer"
cagacgtgtgctcttccgatctatgtaaaccattgctgtgccatt

SEQ ID NO: 524 - DNA, 20 bp, Artificial Sequence
  source: /note="Description of Artificial Sequence: Synthetic primer"
ccagttcttcctgacaccgg

SEQ ID NO: 525 - DNA, 43 bp, Artificial Sequence
  source: /note="Description of Artificial Sequence: Synthetic primer"
cagacgtgtgctcttccgatctccaaagtttgcagcctatacc

SEQ ID NO: 526 - DNA, 20 bp, Artificial Sequence
  source: /note="Description of Artificial Sequence: Synthetic primer"
accaaccagaccaggactta

SEQ ID NO: 527 - DNA, 43 bp, Artificial Sequence
  source: /note="Description of Artificial Sequence: Synthetic primer"
cagacgtgtgctcttccgatcttcactaggagacgtggaattg

SEQ ID NO: 528 - DNA, 19 bp, Artificial Sequence
  source: /note="Description of Artificial Sequence: Synthetic primer"
cacccgtccagaccttgtt

SEQ ID NO: 529 - DNA, 47 bp, Artificial Sequence
  source: /note="Description of Artificial Sequence: Synthetic primer"
cagacgtgtgctcttccgatcttgttttcctcttaacgttagaccac

SEQ ID NO: 530 - DNA, 21 bp, Artificial Sequence
  source: /note="Description of Artificial Sequence: Synthetic primer"
tgcaagagtgacagtggattg

SEQ ID NO: 531 - DNA, 46 bp, Artificial Sequence
  source: /note="Description of Artificial Sequence: Synthetic primer"
cagacgtgtgctcttccgatctgctgatattctgcaacactgtaca

SEQ ID NO: 532 - DNA, 19 bp, Artificial Sequence
  source: /note="Description of Artificial Sequence: Synthetic primer"
tgtcctcacggtgcctttt

SEQ ID NO: 533 - DNA, 42 bp, Artificial Sequence
  source: /note="Description of Artificial Sequence: Synthetic primer"
cagacgtgtgctcttccgatctgtaggcagacacagggactt

SEQ ID NO: 534 - DNA, 21 bp, Artificial Sequence
  source: /note="Description of Artificial Sequence: Synthetic primer"
cctcaagggggactgtctttc

SEQ ID NO: 535 - DNA, 42 bp, Artificial Sequence
  source: /note="Description of Artificial Sequence: Synthetic primer"
cagacgtgtgctcttccgatctgcatatcctgagccatcggt

SEQ ID NO: 536 - DNA, 20 bp, Artificial Sequence
  source: /note="Description of Artificial Sequence: Synthetic primer"
attgctggtagagaccccca

SEQ ID NO: 537 - DNA, 40 bp, Artificial Sequence
  source: /note="Description of Artificial Sequence: Synthetic primer"
cagacgtgtgctcttccgatctcccccatttccccgatgt

SEQ ID NO: 538 - DNA, 20 bp, Artificial Sequence
  source: /note="Description of Artificial Sequence: Synthetic primer"
cccagccagctgtggtattc

SEQ ID NO: 539 - DNA, 42 bp, Artificial Sequence
  source: /note="Description of Artificial Sequence: Synthetic primer"
cagacgtgtgctcttccgatcttggaactgaactgagctgct

SEQ ID NO: 540 - DNA, 20 bp, Artificial Sequence
  source: /note="Description of Artificial Sequence: Synthetic primer"
ctaggcagccaacctaagca

SEQ ID NO: 541 - DNA, 42 bp, Artificial Sequence
  source: /note="Description of Artificial Sequence: Synthetic primer"
cagacgtgtgctcttccgatctcctgcaatctgagccagtgc

SEQ ID NO: 542 - DNA, 20 bp, Artificial Sequence
  source: /note="Description of Artificial Sequence: Synthetic primer"
agtggaccttaggccttcct

SEQ ID NO: 543 - DNA, 43 bp, Artificial Sequence
  source: /note="Description of Artificial Sequence: Synthetic primer"
cagacgtgtgctcttccgatctggctcagacatgttttccgtg

SEQ ID NO: 544 - DNA, 21 bp, Artificial Sequence
  source: /note="Description of Artificial Sequence: Synthetic primer"
tcacttaagacccagggactt

SEQ ID NO: 545 - DNA, 45 bp, Artificial Sequence
  source: /note="Description of Artificial Sequence: Synthetic primer"
cagacgtgtgctcttccgatctaagcatcatctcaacactgactt

SEQ ID NO: 546 - DNA, 20 bp, Artificial Sequence
  source: /note="Description of Artificial Sequence: Synthetic primer"
accatgagaaggacactcgc

SEQ ID NO: 547 - DNA, 42 bp, Artificial Sequence
  source: /note="Description of Artificial Sequence: Synthetic primer"
cagacgtgtgctcttccgatctcgggcttgaattcctgtcct

SEQ ID NO: 548 - DNA, 19 bp, Artificial Sequence
  source: /note="Description of Artificial Sequence: Synthetic primer"
cggcaaatgtagcatgggc

SEQ ID NO: 549 - DNA, 43 bp, Artificial Sequence
  source: /note="Description of Artificial Sequence: Synthetic primer"
cagacgtgtgctcttccgatctggaaagtggctatgcagtttg

SEQ ID NO: 550 - DNA, 21 bp, Artificial Sequence
  source: /note="Description of Artificial Sequence: Synthetic primer"
ggcatcctccacaatagcaga

SEQ ID NO: 551 - DNA, 43 bp, Artificial Sequence
  source: /note="Description of Artificial Sequence: Synthetic primer"
cagacgtgtgctcttccgatctgcattttggtccaagttgtgc

SEQ ID NO: 552 - DNA, 20 bp, Artificial Sequence
  source: /note="Description of Artificial Sequence: Synthetic primer"
cttaaagcccgcctgacaga

SEQ ID NO: 553 - DNA, 42 bp, Artificial Sequence
  source: /note="Description of Artificial Sequence: Synthetic primer"
cagacgtgtgctcttccgatctacattctgatgagcaaccgc

SEQ ID NO: 554 - DNA, 20 bp, Artificial Sequence
  source: /note="Description of Artificial Sequence: Synthetic primer"
acagacgactttgagcctcg

SEQ ID NO: 555 - DNA, 42 bp, Artificial Sequence
  source: /note="Description of Artificial Sequence: Synthetic primer"
cagacgtgtgctcttccgatctatttcaccttttcctgcggc

SEQ ID NO: 556 - DNA, 20 bp, Artificial Sequence
  source: /note="Description of Artificial Sequence: Synthetic primer"
ggagccaagggttcagagac

SEQ ID NO: 557 - DNA, 42 bp, Artificial Sequence
  source: /note="Description of Artificial Sequence: Synthetic primer"
cagacgtgtgctcttccgatcttgctacctcactggggtcct

SEQ ID NO: 558 - DNA, 20 bp, Artificial Sequence
  source: /note="Description of Artificial Sequence: Synthetic primer"
ggccatctcttcctttcgga

SEQ ID NO: 559 - DNA, 41 bp, Artificial Sequence
  source: /note="Description of Artificial Sequence: Synthetic primer"
cagacgtgtgctcttccgatctgtgtgggaactctgccgtg

SEQ ID NO: 560 - DNA, 21 bp, Artificial Sequence
  source: /note="Description of Artificial Sequence: Synthetic primer"
ctcaccccatcatccctttcc

SEQ ID NO: 561 - DNA, 42 bp, Artificial Sequence
  source: /note="Description of Artificial Sequence: Synthetic primer"
cagacgtgtgctcttccgatctgcccagtgagactgtgttgt

SEQ ID NO: 562 - DNA, 20 bp, Artificial Sequence
  source: /note="Description of Artificial Sequence: Synthetic primer"
tactgacggcatgttaggtg

SEQ ID NO: 563 - DNA, 42 bp, Artificial Sequence
  source: /note="Description of Artificial Sequence: Synthetic primer"
cagacgtgtgctcttccgatcttgtgtgtggagtgggatgtg

SEQ ID NO: 564 - DNA, 20 bp, Artificial Sequence
  source: /note="Description of Artificial Sequence: Synthetic primer"
aggcagggaggggactattt

SEQ ID NO: 565 - DNA, 42 bp, Artificial Sequence
  source: /note="Description of Artificial Sequence: Synthetic primer"
cagacgtgtgctcttccgatctggagaaacagagacaggccc

SEQ ID NO: 566 - DNA, 19 bp, Artificial Sequence
  source: /note="Description of Artificial Sequence: Synthetic primer"
gcagtgagaatgagggcca

SEQ ID NO: 567 - DNA, 42 bp, Artificial Sequence
  source: /note="Description of Artificial Sequence: Synthetic primer"
cagacgtgtgctcttccgatctaggcatactgacactttgcc

SEQ ID NO: 568 - DNA, 20 bp, Artificial Sequence
  source: /note="Description of Artificial Sequence: Synthetic primer"
agccagtccaggagtgagac

SEQ ID NO: 569 - DNA, 42 bp, Artificial Sequence
  source: /note="Description of Artificial Sequence: Synthetic primer"
cagacgtgtgctcttccgatctggccacactgaccctgatac

SEQ ID NO: 570 - DNA, 20 bp, Artificial Sequence
  source: /note="Description of Artificial Sequence: Synthetic primer"
cccaaggtcaagatcgccac

SEQ ID NO: 571 - DNA, 42 bp, Artificial Sequence
  source: /note="Description of Artificial Sequence: Synthetic primer"
cagacgtgtgctcttccgatctctgccagctccagaagatgt

SEQ ID NO: 572 - DNA, 21 bp, Artificial Sequence
  source: /note="Description of Artificial Sequence: Synthetic primer"
tgggaagccaaactccatcat

SEQ ID NO: 573 - DNA, 43 bp, Artificial Sequence
  source: /note="Description of Artificial Sequence: Synthetic primer"
cagacgtgtgctcttccgatctggaaaccaatgccacttttgt

SEQ ID NO: 574 - DNA, 21 bp, Artificial Sequence
  source: /note="Description of Artificial Sequence: Synthetic primer"
gccttcaagactgaacaccga

SEQ ID NO: 575 - DNA, 43 bp, Artificial Sequence
  source: /note="Description of Artificial Sequence: Synthetic primer"
cagacgtgtgctcttccgatctgcccctcagagatcaacagac

SEQ ID NO: 576 - DNA, 20 bp, Artificial Sequence
  source: /note="Description of Artificial Sequence: Synthetic primer"
ttggagaaggtgctggtgac

SEQ ID NO: 577 - DNA, 42 bp, Artificial Sequence
  source: /note="Description of Artificial Sequence: Synthetic primer"
cagacgtgtgctcttccgatctcttacccagtgctctgcaac

SEQ ID NO: 578 - DNA, 20 bp, Artificial Sequence
  source: /note="Description of Artificial Sequence: Synthetic primer"
tattcctttgcccggcatca

SEQ ID NO: 579 - DNA, 42 bp, Artificial Sequence
  source: /note="Description of Artificial Sequence: Synthetic primer"
cagacgtgtgctcttccgatctaccttgggcactgttgaagt

SEQ ID NO: 580 - DNA, 20 bp, Artificial Sequence
  source: /note="Description of Artificial Sequence: Synthetic primer"
acttgcacatcatggagggt

SEQ ID NO: 581 - DNA, 47 bp, Artificial Sequence
  source: /note="Description of Artificial Sequence: Synthetic primer"
cagacgtgtgctcttccgatcttccataagctattttggtttagtgc

SEQ ID NO: 582 - DNA, 20 bp, Artificial Sequence
  source: /note="Description of Artificial Sequence: Synthetic primer"
ggtccctccaaaccgttgtc

SEQ ID NO: 583 - DNA, 44 bp, Artificial Sequence
  source: /note="Description of Artificial Sequence: Synthetic primer"
cagacgtgtgctcttccgatctgaactagggagggggaaagaag

SEQ ID NO: 584 - DNA, 20 bp, Artificial Sequence
  source: /note="Description of Artificial Sequence: Synthetic primer"
tgggagttgatcgcctttcc

SEQ ID NO: 585 - DNA, 43 bp, Artificial Sequence
  source: /note="Description of Artificial Sequence: Synthetic primer"
cagacgtgtgctcttccgatctctcattctgaaggagccccat

SEQ ID NO: 586 - DNA, 20 bp, Artificial Sequence
  source: /note="Description of Artificial Sequence: Synthetic primer"
tggactggttgttgccaaac

SEQ ID NO: 587 - DNA, 42 bp, Artificial Sequence
  source: /note="Description of Artificial Sequence: Synthetic primer"
cagacgtgtgctcttccgatctctctgagagttcccctgtcc

SEQ ID NO: 588 - DNA, 20 bp, Artificial Sequence
  source: /note="Description of Artificial Sequence: Synthetic primer"
ttcctcctcatcaccatcgc

SEQ ID NO: 589 - DNA, 42 bp, Artificial Sequence
  source: /note="Description of Artificial Sequence: Synthetic primer"
cagacgtgtgctcttccgatctcttaccacccctcagagtgc

SEQ ID NO: 590 - DNA, 20 bp, Artificial Sequence
  source: /note="Description of Artificial Sequence: Synthetic primer"
gaagctgaatgcctgagggg

SEQ ID NO: 591 - DNA, 41 bp, Artificial Sequence
  source: /note="Description of Artificial Sequence: Synthetic primer"
cagacgtgtgctcttccgatctgtcccatctgctatgccca

SEQ ID NO: 592 - DNA, 20 bp, Artificial Sequence
  source: /note="Description of Artificial Sequence: Synthetic primer"
gagtgctgcctggagtactt

SEQ ID NO: 593 - DNA, 42 bp, Artificial Sequence
  source: /note="Description of Artificial Sequence: Synthetic primer"
cagacgtgtgctcttccgatctctcaccccagactcctgact

SEQ ID NO: 594 - DNA, 20 bp, Artificial Sequence
  source: /note="Description of Artificial Sequence: Synthetic primer"
gctatggtgagccgtgattg

SEQ ID NO: 595 - DNA, 42 bp, Artificial Sequence
  source: /note="Description of Artificial Sequence: Synthetic primer"
cagacgtgtgctcttccgatcttcctcacccccacctctcta

SEQ ID NO: 596 - DNA, 20 bp, Artificial Sequence
  source: /note="Description of Artificial Sequence: Synthetic primer"
gacctcagaggcctcctact

SEQ ID NO: 597 - DNA, 41 bp, Artificial Sequence
  source: /note="Description of Artificial Sequence: Synthetic primer"
cagacgtgtgctcttccgatctccaatatcctcgctcccgg

SEQ ID NO: 598 - DNA, 20 bp, Artificial Sequence
  source: /note="Description of Artificial Sequence: Synthetic primer"
ttcaggactccctccagcat

SEQ ID NO: 599 - DNA, 42 bp, Artificial Sequence
  source: /note="Description of Artificial Sequence: Synthetic primer"
cagacgtgtgctcttccgatctaggtaccaaatgcctgtgcc

SEQ ID NO: 600 - DNA, 20 bp, Artificial Sequence
  source: /note="Description of Artificial Sequence: Synthetic primer"
tgaacttcagggagggtggt

SEQ ID NO: 601 - DNA, 42 bp, Artificial Sequence
  source: /note="Description of Artificial Sequence: Synthetic primer"
cagacgtgtgctcttccgatcttcctcgtatgcatggaaccc

SEQ ID NO: 602 - DNA, 20 bp, Artificial Sequence
  source: /note="Description of Artificial Sequence: Synthetic primer"
ccaaagggaagagtgcaggg

SEQ ID NO: 603 - DNA, 49 bp, Artificial Sequence
  source: /note="Description of Artificial Sequence: Synthetic primer"
cagacgtgtgctcttccgatctattctgtataacactcatatctttgcc

SEQ ID NO: 604 - DNA, 21 bp, Artificial Sequence
  source: /note="Description of Artificial Sequence: Synthetic primer"
agaatcattaggccaggcgtg

SEQ ID NO: 605 - DNA, 43 bp, Artificial Sequence
  source: /note="Description of Artificial Sequence: Synthetic primer"
cagacgtgtgctcttccgatctctggccaatatgctgaaaccc

SEQ ID NO: 606 - DNA, 20 bp, Artificial Sequence
  source: /note="Description of Artificial Sequence: Synthetic primer"
atttgaggctgcagtgagct

SEQ ID NO: 607 - DNA, 42 bp, Artificial Sequence
  source: /note="Description of Artificial Sequence: Synthetic primer"
cagacgtgtgctcttccgatctagacaagagctggctcacct

SEQ ID NO: 608 - DNA, 20 bp, Artificial Sequence
  source: /note="Description of Artificial Sequence: Synthetic primer"
cctccccagcctttgatcag

SEQ ID NO: 609 - DNA, 42 bp, Artificial Sequence
  source: /note="Description of Artificial Sequence: Synthetic primer"
cagacgtgtgctcttccgatcttcctcgcaagctgggtaatc

SEQ ID NO: 610 - DNA, 20 bp, Artificial Sequence
  source: /note="Description of Artificial Sequence: Synthetic primer"
ccagcaccagggagtttcta

SEQ ID NO: 611 - DNA, 42 bp, Artificial Sequence
  source: /note="Description of Artificial Sequence: Synthetic primer"
cagacgtgtgctcttccgatctacagcatgtcacaaggctgt

SEQ ID NO: 612 - DNA, 20 bp, Artificial Sequence
  source: /note="Description of Artificial Sequence: Synthetic primer"
aggcagatggaacttgagcc

SEQ ID NO: 613 - DNA, 44 bp, Artificial Sequence
  source: /note="Description of Artificial Sequence: Synthetic primer"
cagacgtgtgctcttccgatctgcattcgaagatccccagactt

SEQ ID NO: 614 - DNA, 20 bp, Artificial Sequence
  source: /note="Description of Artificial Sequence: Synthetic primer"
tccccatcgtcctccttgtc

SEQ ID NO: 615 - DNA, 41 bp, Artificial Sequence
  source: /note="Description of Artificial Sequence: Synthetic primer"
cagacgtgtgctcttccgatctttgccggctctccagagta

SEQ ID NO: 616 - DNA, 24 bp, Artificial Sequence
  source: /note="Description of Artificial Sequence: Synthetic primer"
gttcccatgttaaatcccattcat

SEQ ID NO: 617 - DNA, 47 bp, Artificial Sequence
  source: /note="Description of Artificial Sequence: Synthetic primer"
cagacgtgtgctcttccgatcttaccaggaatggatgtcgctaatca

SEQ ID NO: 618 - DNA, 20 bp, Artificial Sequence
  source: /note="Description of Artificial Sequence: Synthetic primer"
accctctctccctccctttc

SEQ ID NO: 619 - DNA, 42 bp, Artificial Sequence; identical to SEQ ID NO: 379
  source: /note="Description of Artificial Sequence: Synthetic primer"

SEQ ID NO: 620 - DNA, 20 bp, Artificial Sequence
  source: /note="Description of Artificial Sequence: Synthetic primer"
ccccaaccacttcattcttg

SEQ ID NO: 621 - DNA, 43 bp, Artificial Sequence; identical to SEQ ID NO: 51
  source: /note="Description of Artificial Sequence: Synthetic primer"

SEQ ID NO: 622 - DNA, 20 bp, Artificial Sequence
  source: /note="Description of Artificial Sequence: Synthetic primer"
cctcccccagtctctcttct

SEQ ID NO: 623 - DNA, 42 bp, Artificial Sequence; identical to SEQ ID NO: 147
  source: /note="Description of Artificial Sequence: Synthetic primer"

SEQ ID NO: 624 - DNA, 20 bp, Artificial Sequence
  source: /note="Description of Artificial Sequence: Synthetic primer"
ctgcctcggtgagttttctc

SEQ ID NO: 625 - DNA, 20 bp, Artificial Sequence
  source: /note="Description of Artificial Sequence: Synthetic primer"
cttcccgttacggttttgac

SEQ ID NO: 626 - DNA, 20 bp, Artificial Sequence
  source: /note="Description of Artificial Sequence: Synthetic primer"
aaaaccggattaggccatta

SEQ ID NO: 627 - DNA, 20 bp, Artificial Sequence
  source: /note="Description of Artificial Sequence: Synthetic primer"
tctcgtcatgaccgaaaaag

SEQ ID NO: 628 - DNA, 20 bp, Artificial Sequence
  source: /note="Description of Artificial Sequence: Synthetic primer"
caacgcctacaaaagccagt

SEQ ID NO: 629 - DNA, 20 bp, Artificial Sequence
  source: /note="Description of Artificial Sequence: Synthetic primer"
gtggcaaagcaaaagttcaa

SEQ ID NO: 630 - DNA, 22 bp, Artificial Sequence
  source: /note="Description of Artificial Sequence: Synthetic primer"
tgagaaagcgtttgatgatgta

SEQ ID NO: 631 - DNA, 20 bp, Artificial Sequence
  source: /note="Description of Artificial Sequence: Synthetic primer"
gccagtttatcccgtcaaag

SEQ ID NO: 632 - DNA, 20 bp, Artificial Sequence
  source: /note="Description of Artificial Sequence: Synthetic primer"
cttcccgttacggttttgac

SEQ ID NO: 633 - DNA, 20 bp, Artificial Sequence
  source: /note="Description of Artificial Sequence: Synthetic primer"
aaaaccggattaggccatta

SEQ ID NO: 634 - DNA, 20 bp, Artificial Sequence
  source: /note="Description of Artificial Sequence: Synthetic primer"
tctcgtcatgaccgaaaaag

SEQ ID NO: 635 - DNA, 20 bp, Artificial Sequence
  source: /note="Description of Artificial Sequence: Synthetic primer"
caacgcctacaaaagccagt

SEQ ID NO: 636 - DNA, 20 bp, Artificial Sequence
  source: /note="Description of Artificial Sequence: Synthetic primer"
ttgactttgccttggagagc

SEQ ID NO: 637 - DNA, 24 bp, Artificial Sequence
  source: /note="Description of Artificial Sequence: Synthetic primer"
tttttcttacagtgtcttggcata

SEQ ID NO: 638 - DNA, 19 bp, Artificial Sequence
  source: /note="Description of Artificial Sequence: Synthetic primer"
cgtgaccctaagcgaggag

SEQ ID NO: 639 - DNA, 21 bp, Artificial Sequence
  source: /note="Description of Artificial Sequence: Synthetic primer"
tttgcagtgatttgaagacca

SEQ ID NO: 640 - DNA, 20 bp, Artificial Sequence
  source: /note="Description of Artificial Sequence: Synthetic primer"
ggcattccttcttctggtca

SEQ ID NO: 641 - DNA, 23 bp, Artificial Sequence
  source: /note="Description of Artificial Sequence: Synthetic primer"
ctgggctatatacagtcctcaaa

SEQ ID NO: 642 - DNA, 21 bp, Artificial Sequence
  source: /note="Description of Artificial Sequence: Synthetic primer"
ggggtgattatgaccagttga

SEQ ID NO: 643 - DNA, 20 bp, Artificial Sequence
  source: /note="Description of Artificial Sequence: Synthetic primer"
tgcatgatcaaatgcaacct

SEQ ID NO: 644 - DNA, 21 bp, Artificial Sequence
  source: /note="Description of Artificial Sequence: Synthetic primer"
tcttccgaaaaatcctcttcc

SEQ ID NO: 645 - DNA, 19 bp, Artificial Sequence
  source: /note="Description of Artificial Sequence: Synthetic primer"
ctggggtcccagtcctatg

SEQ ID NO: 646 - DNA, 21 bp, Artificial Sequence
  source: /note="Description of Artificial Sequence: Synthetic primer"
tgtactgggaaggcaatttca

SEQ ID NO: 647 - DNA, 18 bp, Artificial Sequence
  source: /note="Description of Artificial Sequence: Synthetic primer"
gagccgctggggttactc

SEQ ID NO: 648 - DNA, 21 bp, Artificial Sequence
  source: /note="Description of Artificial Sequence: Synthetic primer"
cagttagttgctgcacatgga

SEQ ID NO: 649 - DNA, 20 bp, Artificial Sequence
  source: /note="Description of Artificial Sequence: Synthetic primer"
ttgcatttcttttggggaag

SEQ ID NO: 650 - DNA, 20 bp, Artificial Sequence
  source: /note="Description of Artificial Sequence: Synthetic primer"
gtcatgcatgcagatggaag

SEQ ID NO: 651 - DNA, 20 bp, Artificial Sequence
  source: /note="Description of Artificial Sequence: Synthetic primer"
gctgcagtgagctgtgatgt

SEQ ID NO: 652 - DNA, 19 bp, Artificial Sequence
  source: /note="Description of Artificial Sequence: Synthetic primer"
gttcctctccgagctcacc

SEQ ID NO: 653 - DNA, 20 bp, Artificial Sequence
  source: /note="Description of Artificial Sequence: Synthetic primer"
tccgaaagtttccaattcca

SEQ ID NO: 654 - DNA, 21 bp, Artificial Sequence
  source: /note="Description of Artificial Sequence: Synthetic primer"
ttgtttgggagactctgcatt

SEQ ID NO: 655 - DNA, 20 bp, Artificial Sequence
  source: /note="Description of Artificial Sequence: Synthetic primer"
gaccccacttggactggtag

SEQ ID NO: 656 - DNA, 20 bp, Artificial Sequence
  source: /note="Description of Artificial Sequence: Synthetic primer"
gtgatcttgattgcggcttt

SEQ ID NO: 657 - DNA, 20 bp, Artificial Sequence
  source: /note="Description of Artificial Sequence: Synthetic primer"
gggggaaaaactacaagtgc

SEQ ID NO: 658 - DNA, 20 bp, Artificial Sequence
  source: /note="Description of Artificial Sequence: Synthetic primer"
tgattccttttcctgcctgt

SEQ ID NO: 659 - DNA, 20 bp, Artificial Sequence
  source: /note="Description of Artificial Sequence: Synthetic primer"
aaaaacctccaggccagact

SEQ ID NO: 660 - DNA, 20 bp, Artificial Sequence
  source: /note="Description of Artificial Sequence: Synthetic primer"
aatcaaaataacgccccaga

SEQ ID NO: 661 - DNA, 20 bp, Artificial Sequence
  source: /note="Description of Artificial Sequence: Synthetic primer"
ttgctaaaaattggcagagc

SEQ ID NO: 662 - DNA, 22 bp, Artificial Sequence
  source: /note="Description of Artificial Sequence: Synthetic primer"
ttgttaagtgccaaacaaagga

SEQ ID NO: 663 - DNA, 19 bp, Artificial Sequence
  source: /note="Description of Artificial Sequence: Synthetic primer"
aagctgggaagagcaaagc

SEQ ID NO: 664 - DNA, 19 bp, Artificial Sequence
  source: /note="Description of Artificial Sequence: Synthetic primer"
aggacagagggtggtcgtc

SEQ ID NO: 665 - DNA, 21 bp, Artificial Sequence
  source: /note="Description of Artificial Sequence: Synthetic primer"
tgagtgctgtctccatgtttg

SEQ ID NO: 666 - DNA, 22 bp, Artificial Sequence
  source: /note="Description of Artificial Sequence: Synthetic primer"
cctcacagctgttgctgttatt

SEQ ID NO: 667 - DNA, 20 bp, Artificial Sequence
  source: /note="Description of Artificial Sequence: Synthetic primer"
aaaacacccagctaggacca

SEQ ID NO: 668 - DNA, 20 bp, Artificial Sequence
  source: /note="Description of Artificial Sequence: Synthetic primer"
aactgaggcacgagcaaagt

SEQ ID NO: 669 - DNA, 20 bp, Artificial Sequence
  source: /note="Description of Artificial Sequence: Synthetic primer"
gctttatgggtggatgctga

SEQ ID NO: 670 - DNA, 20 bp, Artificial Sequence
  source: /note="Description of Artificial Sequence: Synthetic primer"
ataatatcgccagcctcagc

SEQ ID NO: 671 - DNA, 20 bp, Artificial Sequence
  source: /note="Description of Artificial Sequence: Synthetic primer"
tccagagtgtgctggatgac

SEQ ID NO: 672 - DNA, 20 bp, Artificial Sequence
  source: /note="Description of Artificial Sequence: Synthetic primer"
tgcaagccatttatgggaat

SEQ ID NO: 673 - DNA, 25 bp, Artificial Sequence
  source: /note="Description of Artificial Sequence: Synthetic primer"
tggaatgaggtctcttagtacagtt

SEQ ID NO: 674 - DNA, 21 bp, Artificial Sequence
  source: /note="Description of Artificial Sequence: Synthetic primer"
tcccagaaacacctgtaagga

SEQ ID NO: 675 - DNA, 20 bp, Artificial Sequence
  source: /note="Description of Artificial Sequence: Synthetic primer"
tgtctaggcaggacctgtgg

SEQ ID NO: 676 - DNA, 20 bp, Artificial Sequence
  source: /note="Description of Artificial Sequence: Synthetic primer"
agtgatgctgcgactcacac

SEQ ID NO: 677 - DNA, 22 bp, Artificial Sequence
  source: /note="Description of Artificial Sequence: Synthetic primer"
ggctcagaaagtctctctttcc

SEQ ID NO: 678 - DNA, 20 bp, Artificial Sequence
  source: /note="Description of Artificial Sequence: Synthetic primer"
ctcccaaactcaggctttca

SEQ ID NO: 679 - DNA, 19 bp, Artificial Sequence
  source: /note="Description of Artificial Sequence: Synthetic primer"
aaagcgctgggattacagg

SEQ ID NO: 680 - DNA, 20 bp, Artificial Sequence
  source: /note="Description of Artificial Sequence: Synthetic primer"
cgtccagttgcttggagaag

SEQ ID NO: 681 - DNA, 20 bp, Artificial Sequence
  source: /note="Description of Artificial Sequence: Synthetic primer"
aataaccttggctgccgtct

SEQ ID NO: 682 - DNA, 20 bp, Artificial Sequence
  source: /note="Description of Artificial Sequence: Synthetic primer"
gggaattctcagtgccaact

SEQ ID NO: 683 - DNA, 20 bp, Artificial Sequence
  source: /note="Description of Artificial Sequence: Synthetic primer"
gcatcctgggctacactgag

SEQ ID NO: 684 - DNA, 23 bp, Artificial Sequence
  source: /note="Description of Artificial Sequence: Synthetic primer"
tgctgggaacaatgactataaga

SEQ ID NO: 685 - DNA, 21 bp, Artificial Sequence
  source: /note="Description of Artificial Sequence: Synthetic primer"
gcctaaaacactttgggtggt

SEQ ID NO: 686 - DNA, 20 bp, Artificial Sequence
  source: /note="Description of Artificial Sequence: Synthetic primer"
gggtgcccacaaaatagaga

SEQ ID NO: 687 - DNA, 20 bp, Artificial Sequence
  source: /note="Description of Artificial Sequence: Synthetic primer"
gagactgggtctcgctttgt

SEQ ID NO: 688 - DNA, 20 bp, Artificial Sequence
  source: /note="Description of Artificial Sequence: Synthetic primer"
tggggaaggctttctctagg

SEQ ID NO: 689 - DNA, 23 bp, Artificial Sequence
  source: /note="Description of Artificial Sequence: Synthetic primer"
ttcaacttgagtgatctgagctg

SEQ ID NO: 690 - DNA, 20 bp, Artificial Sequence
  source: /note="Description of Artificial Sequence: Synthetic primer"
tatgggcaaccctaaggtga

SEQ ID NO: 691 - DNA, 20 bp, Artificial Sequence
  source: /note="Description of Artificial Sequence: Synthetic primer"
cgctgcgacactacatcaac

SEQ ID NO: 692 - DNA, 20 bp, Artificial Sequence
  source: /note="Description of Artificial Sequence: Synthetic primer"
tggagtcttgctctgtcacc

SEQ ID NO: 693 - DNA, 19 bp, Artificial Sequence
  source: /note="Description of Artificial Sequence: Synthetic primer"
acgaggtgaaggagcaggt

SEQ ID NO: 694 - DNA, 20 bp, Artificial Sequence
  source: /note="Description of Artificial Sequence: Synthetic primer"
cgatgcctttgggtagagag

SEQ ID NO: 695 - DNA, 20 bp, Artificial Sequence
  source: /note="Description of Artificial Sequence: Synthetic primer"
actgatcgtccaaggactgg

SEQ ID NO: 696 - DNA, 27 bp, Artificial Sequence
  source: /note="Description of Artificial Sequence: Synthetic primer"
aaaaagaaatctggtcttgttagaaaa

SEQ ID NO: 697 - DNA, 24 bp, Artificial Sequence
  source: /note="Description of Artificial Sequence: Synthetic primer"
ttgaaaagtggtaaggaattgtga

SEQ ID NO: 698 - DNA, 23 bp, Artificial Sequence
  source: /note="Description of Artificial Sequence: Synthetic primer"
caccaagaattgattttgtagcc

SEQ ID NO: 699 - DNA, 20 bp, Artificial Sequence
  source: /note="Description of Artificial Sequence: Synthetic primer"
aaaaatgggggaaaatggtg

SEQ ID NO: 700 - DNA, 20 bp, Artificial Sequence
  source: /note="Description of Artificial Sequence: Synthetic primer"
catggttgaaaccccatctc

SEQ ID NO: 701 - DNA, 20 bp, Artificial Sequence
  source: /note="Description of Artificial Sequence: Synthetic primer"
ttcaaagcctccacgactct

SEQ ID NO: 702 - DNA, 20 bp, Artificial Sequence
  source: /note="Description of Artificial Sequence: Synthetic primer"
gctggaacaggtgcctaaag

SEQ ID NO: 703 - DNA, 20 bp, Artificial Sequence
  source: /note="Description of Artificial Sequence: Synthetic primer"
ccctaagggaacgacactca

SEQ ID NO: 704 - DNA, 19 bp, Artificial Sequence
  source: /note="Description of Artificial Sequence: Synthetic primer"
acctgctacaagccctgga

SEQ ID NO: 705 - DNA, 20 bp, Artificial Sequence
  source: /note="Description of Artificial Sequence: Synthetic primer"
ggatccctaagaccgtggag

SEQ ID NO: 706 - DNA, 18 bp, Artificial Sequence
  source: /note="Description of Artificial Sequence: Synthetic primer"
ccacctcagaggctccaa

SEQ ID NO: 707 - DNA, 27 bp, Artificial Sequence
  source: /note="Description of Artificial Sequence: Synthetic primer"
tgctgtattttaaaagaatgattatga

SEQ ID NO: 708 - DNA, 20 bp, Artificial Sequence
  source: /note="Description of Artificial Sequence: Synthetic primer"
gtagctgggacgctggttta

SEQ ID NO: 709 - DNA, 20 bp, Artificial Sequence
  source: /note="Description of Artificial Sequence: Synthetic primer"
attcccttccccctacaaga

SEQ ID NO: 710 - DNA, 20 bp, Artificial Sequence
  source: /note="Description of Artificial Sequence: Synthetic primer"
cctgagtgcaacgacatcac

SEQ ID NO: 711 - DNA, 18 bp, Artificial Sequence
  source: /note="Description of Artificial Sequence: Synthetic primer"
gggggaaccagcagaaat

SEQ ID NO: 712 - DNA, 18 bp, Artificial Sequence
  source: /note="Description of Artificial Sequence: Synthetic primer"
gacctagggcgagggttc

SEQ ID NO: 713 - DNA, 20 bp, Artificial Sequence
  source: /note="Description of Artificial Sequence: Synthetic primer"
aattcctgaagccagatcca

SEQ ID NO: 714 - DNA, 25 bp, Artificial Sequence
  source: /note="Description of Artificial Sequence: Synthetic primer"
aaaatgtttattgttgtagctctgg

SEQ ID NO: 715 - DNA, 23 bp, Artificial Sequence
  source: /note="Description of Artificial Sequence: Synthetic primer"
tttcaagagctcaacagatgaca

SEQ ID NO: 716 - DNA, 19 bp, Artificial Sequence
  source: /note="Description of Artificial Sequence: Synthetic primer"
gactgcccggacaagtttt

SEQ ID NO: 717 - DNA, 19 bp, Artificial Sequence
  source: /note="Description of Artificial Sequence: Synthetic primer"
gagaaggtgccccaaaatg

SEQ ID NO: 718 - DNA, 20 bp, Artificial Sequence
  source: /note="Description of Artificial Sequence: Synthetic primer"
agccactggactgacgactt

SEQ ID NO: 719 - DNA, 21 bp, Artificial Sequence
  source: /note="Description of Artificial Sequence: Synthetic primer"
ggaggactagtgagggaggtg

SEQ ID NO: 720 - DNA, 20 bp, Artificial Sequence
  source: /note="Description of Artificial Sequence: Synthetic primer"
ggcaagtgatgtggcaatta

SEQ ID NO: 721 - DNA, 20 bp, Artificial Sequence
  source: /note="Description of Artificial Sequence: Synthetic primer"
gttggagcacctggaaagaa

SEQ ID NO: 722 - DNA, 19 bp, Artificial Sequence
  source: /note="Description of Artificial Sequence: Synthetic primer"
atgcctgcctcaccttcat

SEQ ID NO: 723 - DNA, 19 bp, Artificial Sequence
  source: /note="Description of Artificial Sequence: Synthetic primer"
acaggggcactgtcaacac

SEQ ID NO: 724 - DNA, 22 bp, Artificial Sequence
  source: /note="Description of Artificial Sequence: Synthetic primer"
aaaaatcatgtgttgcagcttt

SEQ ID NO: 725 - DNA, 20 bp, Artificial Sequence
  source: /note="Description of Artificial Sequence: Synthetic primer"
tgctttcacaacatttgcag

SEQ ID NO: 726 - DNA, 20 bp, Artificial Sequence
  source: /note="Description of Artificial Sequence: Synthetic primer"
aatgtttccttgtgcctgct

SEQ ID NO: 727 - DNA, 20 bp, Artificial Sequence
  source: /note="Description of Artificial Sequence: Synthetic primer"
atatcctgagccatcggtga

SEQ ID NO: 728 - DNA, 20 bp, Artificial Sequence
  source: /note="Description of Artificial Sequence: Synthetic primer"
ttttggtaccccaggctatg

SEQ ID NO: 729 - DNA, 20 bp, Artificial Sequence
  source: /note="Description of Artificial Sequence: Synthetic primer"
accccgtggcattacataac

SEQ ID NO: 730 - DNA, 20 bp, Artificial Sequence
  source: /note="Description of Artificial Sequence: Synthetic primer"
cttccaggaggcacagaaat

SEQ ID NO: 731 - DNA, 20 bp, Artificial Sequence
  source: /note="Description of Artificial Sequence: Synthetic primer"
ctaacctgggcgacagagtg

SEQ ID NO: 732 - DNA, 25 bp, Artificial Sequence
  source: /note="Description of Artificial Sequence: Synthetic primer"
atatttggacataacagacttggaa

SEQ ID NO: 733 - DNA, 26 bp, Artificial Sequence
  source: /note="Description of Artificial Sequence: Synthetic primer"
tgctgacttttaaaataagtgattcg

SEQ ID NO: 734 - DNA, 19 bp, Artificial Sequence
  source: /note="Description of Artificial Sequence: Synthetic primer"
gcggcagagtagccctaac

SEQ ID NO: 735 - DNA, 21 bp, Artificial Sequence
  source: /note="Description of Artificial Sequence: Synthetic primer"
tgggctatttctattgctgct

SEQ ID NO: 736 - DNA, 20 bp, Artificial Sequence
  source: /note="Description of Artificial Sequence: Synthetic primer"
aatggaaagtggctatgcag

SEQ ID NO: 737 - DNA, 25 bp, Artificial Sequence
  source: /note="Description of Artificial Sequence: Synthetic primer"
ggttgtagtcactttagatggaaaa

SEQ ID NO: 738 - DNA, 21 bp, Artificial Sequence
  source: /note="Description of Artificial Sequence: Synthetic primer"
tttgtttgactttgagcacca

SEQ ID NO: 739 - DNA, 26 bp, Artificial Sequence
  source: /note="Description of Artificial Sequence: Synthetic primer"
aatgtttctctgtaaatattgccatt

SEQ ID NO: 740 - DNA, 20 bp, Artificial Sequence
  source: /note="Description of Artificial Sequence: Synthetic primer"
cacccccatatggtcatagc

SEQ ID NO: 741 - DNA, 19 bp, Artificial Sequence
  source: /note="Description of Artificial Sequence: Synthetic primer"
agcaccaggtgatcctcag

SEQ ID NO: 742 - DNA, 23 bp, Artificial Sequence
  source: /note="Description of Artificial Sequence: Synthetic primer"
tgttttgctgtaacattgaagga

SEQ ID NO: 743 - DNA, 19 bp, Artificial Sequence
  source: /note="Description of Artificial Sequence: Synthetic primer"
taatgccacagtggggatg

SEQ ID NO: 744 - DNA, 20 bp, Artificial Sequence
  source: /note="Description of Artificial Sequence: Synthetic primer"
gggcctaaactttggcagtt

SEQ ID NO: 745 - DNA, 22 bp, Artificial Sequence
  source: /note="Description of Artificial Sequence: Synthetic primer"
ttttaccttccatggctctttt

SEQ ID NO: 746 - DNA, 23 bp, Artificial Sequence
  source: /note="Description of Artificial Sequence: Synthetic primer"
gccttactctgattcagcctctt

SEQ ID NO: 747 - DNA, 23 bp, Artificial Sequence
  source: /note="Description of Artificial Sequence: Synthetic primer"
cgtaacaaaattcattgtggtgt

SEQ ID NO: 748 - DNA, 20 bp, Artificial Sequence
  source: /note="Description of Artificial Sequence: Synthetic primer"
agaaccgctcctacagcaag

SEQ ID NO: 749 - DNA, 20 bp, Artificial Sequence
  source: /note="Description of Artificial Sequence: Synthetic primer"
gtgctttcttttgtgggaca

SEQ ID NO: 750 - DNA, 20 bp, Artificial Sequence
  source: /note="Description of Artificial Sequence: Synthetic primer"
gggagttctgcatttgatcc

SEQ ID NO: 751 - DNA, 20 bp, Artificial Sequence
  source: /note="Description of Artificial Sequence: Synthetic primer"
tgggtcagaggacttcaagg

SEQ ID NO: 752 - DNA, 21 bp, Artificial Sequence
  source: /note="Description of Artificial Sequence: Synthetic primer"
agggttctgatcacattgcac

SEQ ID NO: 753 - DNA, 20 bp, Artificial Sequence
  source: /note="Description of Artificial Sequence: Synthetic primer"
ctgcaggactggtcgttttt

SEQ ID NO: 754 - DNA, 20 bp, Artificial Sequence
  source: /note="Description of Artificial Sequence: Synthetic primer"
agggcagggtagagagggta

SEQ ID NO: 755 - DNA, 20 bp, Artificial Sequence
  source: /note="Description of Artificial Sequence: Synthetic primer"
ttcttccatgcggagaaatc

SEQ ID NO: 756 - DNA, 20 bp, Artificial Sequence
  source: /note="Description of Artificial Sequence: Synthetic primer"
catggctgaaggaaaccagt

SEQ ID NO: 757 - DNA, 20 bp, Artificial Sequence
  source: /note="Description of Artificial Sequence: Synthetic primer"
ttgccagctatcacatgtcc

SEQ ID NO: 758 - DNA, 23 bp, Artificial Sequence
  source: /note="Description of Artificial Sequence: Synthetic primer"
tcttttcctgtaccaggtttttc

SEQ ID NO: 759 - DNA, 20 bp, Artificial Sequence
  source: /note="Description of Artificial Sequence: Synthetic primer"
tgactgggaacatcttgctg

SEQ ID NO: 760 - DNA, 20 bp, Artificial Sequence
  source: /note="Description of Artificial Sequence: Synthetic primer"
tggcacctgtacccttcttc

SEQ ID NO: 761 - DNA, 22 bp, Artificial Sequence
  source: /note="Description of Artificial Sequence: Synthetic primer"
ttcaatctcttgcactcaaagc

SEQ ID NO: 762 - DNA, 20 bp, Artificial Sequence
  source: /note="Description of Artificial Sequence: Synthetic primer"
tggagtcactgccaagtcat

SEQ ID NO: 763 - DNA, 20 bp, Artificial Sequence
  source: /note="Description of Artificial Sequence: Synthetic primer"
tttgcatgatgtttgtgtgc

SEQ ID NO: 764 - DNA, 20 bp, Artificial Sequence
  source: /note="Description of Artificial Sequence: Synthetic primer"
gcacccactctgctttgact

SEQ ID NO: 765 - DNA, 20 bp, Artificial Sequence
  source: /note="Description of Artificial Sequence: Synthetic primer"
accatgtagccagctttcaa

SEQ ID NO: 766 - DNA, 20 bp, Artificial Sequence
  source: /note="Description of Artificial Sequence: Synthetic primer"
gcaactgggcatgagtacct

SEQ ID NO: 767 - DNA, 19 bp, Artificial Sequence
  source: /note="Description of Artificial Sequence: Synthetic primer"
ccacacccccttcctactc

SEQ ID NO: 768 - DNA, 23 bp, Artificial Sequence
  source: /note="Description of Artificial Sequence: Synthetic primer"
agtctgcttatttccagctgttt

SEQ ID NO: 769 - DNA, 22 bp, Artificial Sequence
  source: /note="Description of Artificial Sequence: Synthetic primer"
tcctgttcaaaagtcaggatga

SEQ ID NO: 770 - DNA, 20 bp, Artificial Sequence
  source: /note="Description of Artificial Sequence: Synthetic primer"
aaatcacaaatcccctgcaa

SEQ ID NO: 771 - DNA, 20 bp, Artificial Sequence
  source: /note="Description of Artificial Sequence: Synthetic primer"
ctgaacattccagagcgtgt

SEQ ID NO: 772 - DNA, 19 bp, Artificial Sequence
  source: /note="Description of Artificial Sequence: Synthetic primer"
cagtgggaccaccctcact

SEQ ID NO: 773 - DNA, 21 bp, Artificial Sequence
  source: /note="Description of Artificial Sequence: Synthetic primer"
tctgtagatgacctggcttgc

SEQ ID NO: 774 - DNA, 20 bp, Artificial Sequence
  source: /note="Description of Artificial Sequence: Synthetic primer"
tcagaaccaagatgccaaca

SEQ ID NO: 775 - DNA, 20 bp, Artificial Sequence
  source: /note="Description of Artificial Sequence: Synthetic primer"
catgacccagcctatggttt

SEQ ID NO: 776 - DNA, 20 bp, Artificial Sequence
  source: /note="Description of Artificial Sequence: Synthetic primer"
acctcctgcaagaagagctg

SEQ ID NO: 777 - DNA, 21 bp, Artificial Sequence
  source: /note="Description of Artificial Sequence: Synthetic primer"
ttgggaggctttgcttatttt

SEQ ID NO: 778 - DNA, 20 bp, Artificial Sequence
  source: /note="Description of Artificial Sequence: Synthetic primer"
ctgggaaacactccttgcat

SEQ ID NO: 779 - DNA, 20 bp, Artificial Sequence
  source: /note="Description of Artificial Sequence: Synthetic primer"
caacgaatttggctacagca

SEQ ID NO: 780 - DNA, 22 bp, Artificial Sequence
  source: /note="Description of Artificial Sequence: Synthetic primer"
caaaggtcataatgctttcagc

SEQ ID NO: 781 - DNA, 22 bp, Artificial Sequence
  source: /note="Description of Artificial Sequence: Synthetic primer"
tttgacgtatcttttcatccaa

SEQ ID NO: 782 - DNA, 21 bp, Artificial Sequence
  source: /note="Description of Artificial Sequence: Synthetic primer"
tgttgttggtttccaaaaagg

SEQ ID NO: 783 - DNA, 20 bp, Artificial Sequence
  source: /note="Description of Artificial Sequence: Synthetic primer"
gccaacttttgcatgttttg

SEQ ID NO: 784 - DNA, 19 bp, Artificial Sequence
  source: /note="Description of Artificial Sequence: Synthetic primer"
cccaagctgatctggtggt

SEQ ID NO: 785 - DNA, 23 bp, Artificial Sequence
  source: /note="Description of Artificial Sequence: Synthetic primer"
tgctgtgaaagaaacaaacattg

SEQ ID NO: 786 - DNA, 20 bp, Artificial Sequence
  source: /note="Description of Artificial Sequence: Synthetic primer"
gcacgtggatcctgagaact

SEQ ID NO: 787 - DNA, 20 bp, Artificial Sequence
  source: /note="Description of Artificial Sequence: Synthetic primer"
ccagcccagagacactgatt

SEQ ID NO: 788 - DNA, 20 bp, Artificial Sequence
  source: /note="Description of Artificial Sequence: Synthetic primer"
cacgcccagctaatttttgt

SEQ ID NO: 789 - DNA, 19 bp, Artificial Sequence
  source: /note="Description of Artificial Sequence: Synthetic primer"
cctggtggaagacatgcag

SEQ ID NO: 790 - DNA, 20 bp, Artificial Sequence
  source: /note="Description of Artificial Sequence: Synthetic primer"
tcacacctgtaatcccagca

SEQ ID NO: 791 - DNA, 20 bp, Artificial Sequence
  source: /note="Description of Artificial Sequence: Synthetic primer"
cagagctccgcctcattagt

SEQ ID NO: 792 - DNA, 22 bp, Artificial Sequence
  source: /note="Description of Artificial Sequence: Synthetic primer"
tccatttcatcattgtttctgc

SEQ ID NO: 793 - DNA, 23 bp, Artificial Sequence
  source: /note="Description of Artificial Sequence: Synthetic primer"
tggtgtttgtaggtcactgaaca

SEQ ID NO: 794 - DNA, 23 bp, Artificial Sequence
  source: /note="Description of Artificial Sequence: Synthetic primer"
aacatggtccattcacctttatg

SEQ ID NO: 795 - DNA, 20 bp, Artificial Sequence
  source: /note="Description of Artificial Sequence: Synthetic primer"
agagcgagactccgtctcaa

SEQ ID NO: 796 - DNA, 20 bp, Artificial Sequence
  source: /note="Description of Artificial Sequence: Synthetic primer"
agtgagctgagattgcacca

SEQ ID NO: 797 - DNA, 20 bp, Artificial Sequence
  source: /note="Description of Artificial Sequence: Synthetic primer"
agacggccttgagtctcagt

SEQ ID NO: 798 - DNA, 18 bp, Artificial Sequence
  source: /note="Description of Artificial Sequence: Synthetic primer"
gggaatcccttcctggtc

SEQ ID NO: 799 - DNA, 20 bp, Artificial Sequence
  source: /note="Description of Artificial Sequence: Synthetic primer"
cttcctgcctttctcagcag

SEQ ID NO: 800 - DNA, 20 bp, Artificial Sequence
  source: /note="Description of Artificial Sequence: Synthetic primer"
tgcaggtgatcaagaagacg

SEQ ID NO: 801 - DNA, 20 bp, Artificial Sequence
  source: /note="Description of Artificial Sequence: Synthetic primer"
ggttttgagcatgggttcat

SEQ ID NO: 802 - DNA, 19 bp, Artificial Sequence
  source: /note="Description of Artificial Sequence: Synthetic primer"
ccagcccactcctatggat

SEQ ID NO: 803 - DNA, 20 bp, Artificial Sequence
  source: /note="Description of Artificial Sequence: Synthetic primer"
aaactgggacaggggagaac

SEQ ID NO: 804 - DNA, 20 bp, Artificial Sequence
  source: /note="Description of Artificial Sequence: Synthetic primer"
tttgggtaggtgacctgctt

SEQ ID NO: 805 - DNA, 21 bp, Artificial Sequence
  source: /note="Description of Artificial Sequence: Synthetic primer"
tcactgaacgaatgagtgctg

SEQ ID NO: 806 - DNA, 19 bp, Artificial Sequence
  source: /note="Description of Artificial Sequence: Synthetic primer"
acgatgtgcaggaccagtg

SEQ ID NO: 807 - DNA, 20 bp, Artificial Sequence
  source: /note="Description of Artificial Sequence: Synthetic primer"
aatttgcactgaaacgtgga

SEQ ID NO: 808 - DNA, 21 bp, Artificial Sequence
  source: /note="Description of Artificial Sequence: Synthetic primer"
ctgttgtggcccattaaagaa

SEQ ID NO: 809 - DNA, 20 bp, Artificial Sequence
  source: /note="Description of Artificial Sequence: Synthetic primer"
ttccctccagcagtggtatt

SEQ ID NO: 810 - DNA, 20 bp, Artificial Sequence
  source: /note="Description of Artificial Sequence: Synthetic primer"
caccaggaaggaagctgttg

SEQ ID NO: 811 - DNA, 21 bp, Artificial Sequence
  source: /note="Description of Artificial Sequence: Synthetic primer"
tttccttgtgttcttccaagc

SEQ ID NO: 812 - DNA, 22 bp, Artificial Sequence
  source: /note="Description of Artificial Sequence: Synthetic primer"
tcgcaggcattactaatctgaa

SEQ ID NO: 813 - DNA, 20 bp, Artificial Sequence
  source: /note="Description of Artificial Sequence: Synthetic primer"
ctctggctggctaactggaa

SEQ ID NO: 814 - DNA, 18 bp, Artificial Sequence
  source: /note="Description of Artificial Sequence: Synthetic primer"
agagccccaccctcagat

SEQ ID NO: 815 - DNA, 21 bp, Artificial Sequence
  source: /note="Description of Artificial Sequence: Synthetic primer"
tgtgcagagttctccatctga

SEQ ID NO: 816 - DNA, 23 bp, Artificial Sequence
  source: /note="Description of Artificial Sequence: Synthetic primer"
tgcctgttacaaatatcaaggaa

SEQ ID NO: 817 - DNA, 20 bp, Artificial Sequence
  source: /note="Description of Artificial Sequence: Synthetic primer"
tttcccttcttgcatccttc

SEQ ID NO: 818 - DNA, 20 bp, Artificial Sequence
  source: /note="Description of Artificial Sequence: Synthetic primer"
tgtgaccactggcattcatt

SEQ ID NO: 819 - DNA, 20 bp, Artificial Sequence
  source: /note="Description of Artificial Sequence: Synthetic primer"
ctcacacacacggcctgtta

SEQ ID NO: 820 - DNA, 23 bp, Artificial Sequence
  source: /note="Description of Artificial Sequence: Synthetic primer"
cacttgaccaatactgaccctct

SEQ ID NO: 821 - DNA, 20 bp, Artificial Sequence
  source: /note="Description of Artificial Sequence: Synthetic primer"
gtgtgtgccctgtaacctga

SEQ ID NO: 822 - DNA, 20 bp, Artificial Sequence
  source: /note="Description of Artificial Sequence: Synthetic primer"
ccacttcccacttgcagtct

SEQ ID NO: 823 - DNA, 21 bp, Artificial Sequence
  source: /note="Description of Artificial Sequence: Synthetic primer"
tgtgtgtgtgtgtgtgtgtgt

SEQ ID NO: 824 - DNA, 20 bp, Artificial Sequence
  source: /note="Description of Artificial Sequence: Synthetic primer"
tctcccatgcattcaaactg

SEQ ID NO: 825 - DNA, 23 bp, Artificial Sequence
  source: /note="Description of Artificial Sequence: Synthetic primer"
tctaagtgttcctcactgacagg

SEQ ID NO: 826 - DNA, 20 bp, Artificial Sequence
  source: /note="Description of Artificial Sequence: Synthetic primer"
tactctgcagcgaagtgcaa

SEQ ID NO: 827 - DNA, 20 bp, Artificial Sequence
  source: /note="Description of Artificial Sequence: Synthetic primer"
ccaagatcacaccattgcac

SEQ ID NO: 828 - DNA, 25 bp, Artificial Sequence
  source: /note="Description of Artificial Sequence: Synthetic primer"
atatttggacataacagacttggaa

SEQ ID NO: 829 - DNA, 18 bp, Artificial Sequence
  source: /note="Description of Artificial Sequence: Synthetic oligonucleotide"
tttttttttttttttttv

SEQ ID NO: 830 - DNA, 10 bp, Artificial Sequence
  source: /note="Description of Artificial Sequence: Synthetic oligonucleotide"
aaaaaaaaaa

SEQ ID NO: 831 - DNA, 31 bp, Artificial Sequence
  source: /note="Description of Artificial Sequence: Synthetic oligonucleotide"
aaaaaaaaaaaaaaaaaaaaaaaaaaaaaaa

SEQ ID NO: 832 - DNA, 17 bp, Artificial Sequence
  source: /note="Description of Artificial Sequence: Synthetic oligonucleotide"
cgactacgacgactacg

SEQ ID NO: 833 - DNA, 18 bp, Artificial Sequence
  source: /note="Description of Artificial Sequence: Synthetic oligonucleotide"
atgatacgactagcggat

SEQ ID NO: 834 - DNA, 38 bp, Artificial Sequence
  source: /note="Description of Artificial Sequence: Synthetic oligonucleotide"
cgactacgacgactacgcgacatcgactacgagtcggt

SEQ ID NO: 835 - DNA, 24 bp, Artificial Sequence
  source: /note="Description of Artificial Sequence: Synthetic oligonucleotide"
aatgctatgatacgactagcggat

SEQ ID NO: 836 - DNA, 62 bp, Artificial Sequence
  source: /note="Description of Artificial Sequence: Synthetic oligonucleotide"
cgactacgacgactacgcgacatcgactacgagtcggtaatgctatgatacgactagcggat

SEQ ID NO: 837 - DNA, 12 bp, Artificial Sequence
  source: /note="Description of Artificial Sequence: Synthetic oligonucleotide"
agcattaccgac

SEQ ID NO: 838 - DNA, 38 bp, Artificial Sequence; identical to SEQ ID NO: 834
  source: /note="Description of Artificial Sequence: Synthetic oligonucleotide"

SEQ ID NO: 839 - DNA, 24 bp, Artificial Sequence
  source: /note="Description of Artificial Sequence: Synthetic oligonucleotide"
atccgctagtcgtatcataccgac

SEQ ID NO: 840 - DNA, 56 bp, Artificial Sequence
  source: /note="Description of Artificial Sequence: Synthetic oligonucleotide"
cgactacgacgactacgcgacatcgactacgagtcggtatgatacgactagcggat

SEQ ID NO: 841 - DNA, 38 bp, Artificial Sequence; identical to SEQ ID NO: 834
  source: /note="Description of Artificial Sequence: Synthetic oligonucleotide"

SEQ ID NO: 842 - RNA, 24 nt, Artificial Sequence
  source: /note="Description of Artificial Sequence: Synthetic oligonucleotide"
auccgcuagucguaucauaccgac

SEQ ID NO: 843 - DNA, 56 bp, Artificial Sequence; identical to SEQ ID NO: 840
  source: /note="Description of Artificial Sequence: Synthetic oligonucleotide"